European Patent Application EP 4 659 808 A2, published December 10, 2025. Title: MULTISPECIFIC BINDING MOLECULES HAVING SPECIFICITY TO DYSTROGLYCAN AND LAMININ-2. Applicant: SANOFI. Application EP. The sequence listing filed with the application follows.

SEQUENCE LISTING (534 sequences)

SEQ ID NO: 1 - protein, 8 aa, synthetic construct
  REGION 1..8: note = Synthetic Construct
GFTFTDSV

SEQ ID NO: 2 - protein, 8 aa, synthetic construct
  REGION 1..8: note = Synthetic Construct
GFTFSSYA

SEQ ID NO: 3 - protein, 8 aa, synthetic construct
  REGION 1..8: note = Synthetic Construct
GYSFSNYW

SEQ ID NO: 4 - protein, 8 aa, synthetic construct
  REGION 1..8: note = Synthetic Construct
GFNIKDTY

SEQ ID NO: 5 - protein, 8 aa, synthetic construct
  REGION 1..8: note = Synthetic Construct
GYTFTTYY

SEQ ID NO: 6 - protein, 8 aa, synthetic construct
  REGION 1..8: note = Synthetic Construct
GFTFSSYG

SEQ ID NO: 7 - protein, 8 aa, synthetic construct
  REGION 1..8: note = Synthetic Construct
GYSFTSYW

SEQ ID NO: 8 - protein, 8 aa, synthetic construct
  REGION 1..8: note = Synthetic Construct
GYSFTSYW

SEQ ID NO: 9 - protein, 8 aa, synthetic construct
  REGION 1..8: note = Synthetic Construct
IYPGSGSI

SEQ ID NO: 10 - protein, 8 aa, synthetic construct
  REGION 1..8: note = Synthetic Construct
IYPGSGNF

SEQ ID NO: 11 - protein, 8 aa, synthetic construct
  REGION 1..8: note = Synthetic Construct
ISGSGGST

SEQ ID NO: 12 - protein, 8 aa, synthetic construct
  REGION 1..8: note = Synthetic Construct
IYPGDSDT

SEQ ID NO: 13 - protein, 8 aa, synthetic construct
  REGION 1..8: note = Synthetic Construct
IDPANGNT

SEQ ID NO: 14 - protein, 8 aa, synthetic construct
  REGION 1..8: note = Synthetic Construct
INPSAGNT

SEQ ID NO: 15 - protein, 8 aa, synthetic construct
  REGION 1..8: note = Synthetic Construct
IWYDGSNK

SEQ ID NO: 16 - protein, 8 aa, synthetic construct
  REGION 1..8: note = Synthetic Construct
IYPGDSDT

SEQ ID NO: 17 - protein, 8 aa, synthetic construct
  REGION 1..8: note = Synthetic Construct
IYPGDSDT

SEQ ID NO: 18 - protein, 6 aa, synthetic construct
  REGION 1..6: note = Synthetic Construct
AMRRSY

SEQ ID NO: 19 - protein, 6 aa, synthetic construct
  REGION 1..6: note = Synthetic Construct
AMRRSS

SEQ ID NO: 20 - protein, 18 aa, synthetic construct
  REGION 1..18: note = Synthetic Construct
ARLGYCSSTSCYLSAFDI

SEQ ID NO: 21 - protein, 13 aa, synthetic construct
  REGION 1..13: note = Synthetic Construct
RVIINGTTSGFDY

SEQ ID NO: 22 - protein, 10 aa, synthetic construct
  REGION 1..10: note = Synthetic Construct
GRSGGNYVGY

SEQ ID NO: 23 - protein, 10 aa, synthetic construct
  REGION 1..10: note = Synthetic Construct
GRSRGNYFDY

SEQ ID NO: 24 - protein, 6 aa, synthetic construct
  REGION 1..6: note = Synthetic Construct
ARELDI

SEQ ID NO: 25 - protein, 13 aa, synthetic construct
  REGION 1..13: note = Synthetic Construct
AREGMVRGALFDY

SEQ ID NO: 26 - protein, 12 aa, synthetic construct
  REGION 1..12: note = Synthetic Construct
ARQLRDYYGMDV

SEQ ID NO: 27 - protein, 12 aa, synthetic construct
  REGION 1..12: note = Synthetic Construct
ARQLRDYYSMDV

SEQ ID NO: 28 - protein, 11 aa, synthetic construct
  REGION 1..11: note = Synthetic Construct
QSIVHSNGNTY

SEQ ID NO: 29 - protein, 11 aa, synthetic construct
  REGION 1..11: note = Synthetic Construct
QTIVHSNSKTY

SEQ ID NO: 30 - protein, 6 aa, synthetic construct
  REGION 1..6: note = Synthetic Construct
QSISSW

SEQ ID NO: 31 - protein, 6 aa, synthetic construct
  REGION 1..6: note = Synthetic Construct
QSVSSN

SEQ ID NO: 32 - protein, 12 aa, synthetic construct
  REGION 1..12: note = Synthetic Construct
QSLLDSGNQKNY

SEQ ID NO: 33 - protein, 10 aa, synthetic construct
  REGION 1..10: note = Synthetic Construct
QSLKSNQKNY

SEQ ID NO: 34 - protein, 6 aa, synthetic construct
  REGION 1..6: note = Synthetic Construct
QDIRND

SEQ ID NO: 35 - protein, 7 aa, synthetic construct
  REGION 1..7: note = Synthetic Construct
QSVSSSY

SEQ ID NO: 36 - protein, 7 aa, synthetic construct
  REGION 1..7: note = Synthetic Construct
QTISSNY

SEQ ID NO: 37 - protein, 7 aa, synthetic construct
  REGION 1..7: note = Synthetic Construct
QSVSSSY

SEQ ID NO: 38-42 - skipped (5 entries)

SEQ ID NO: 43 - protein, 9 aa, synthetic construct
  REGION 1..9: note = Synthetic Construct
FQGSHVPLT

SEQ ID NO: 44 - protein, 9 aa, synthetic construct
  REGION 1..9: note = Synthetic Construct
QQYNSYPLT

SEQ ID NO: 45 - protein, 9 aa, synthetic construct
  REGION 1..9: note = Synthetic Construct
QHYNNLPLT

SEQ ID NO: 46 - protein, 9 aa, synthetic construct
  REGION 1..9: note = Synthetic Construct
QQYYTYPWT

SEQ ID NO: 47 - protein, 9 aa, synthetic construct
  REGION 1..9: note = Synthetic Construct
LQDFNFPFT

SEQ ID NO: 48 - protein, 9 aa, synthetic construct
  REGION 1..9: note = Synthetic Construct
QQDYNLPYT

SEQ ID NO: 49 - protein, 9 aa, synthetic construct
  REGION 1..9: note = Synthetic Construct
QQDYNLPRT

SEQ ID NO: 50 - protein, 9 aa, synthetic construct
  REGION 1..9: note = Synthetic Construct
QQDYNLPRT

SEQ ID NO: 51 - protein, 8 aa, synthetic construct
  REGION 1..8: note = Synthetic Construct
GYTFTSYN

SEQ ID NO: 52 - protein, 8 aa, synthetic construct
  REGION 1..8: note = Synthetic Construct
GFTFSSYT

SEQ ID NO: 53 - protein, 8 aa, synthetic construct
  REGION 1..8: note = Synthetic Construct
GFTFSSYT

SEQ ID NO: 54 - protein, 8 aa, synthetic construct
  REGION 1..8: note = Synthetic Construct
GYSFTSYW

SEQ ID NO: 55 - protein, 8 aa, synthetic construct
  REGION 1..8: note = Synthetic Construct
GFTFDDYG

SEQ ID NO: 56 - protein, 8 aa, synthetic construct
  REGION 1..8: note = Synthetic Construct
INPYNDGT

SEQ ID NO: 57 - protein, 8 aa, synthetic construct
  REGION 1..8: note = Synthetic Construct
ISSGGGNT

SEQ ID NO: 58 - protein, 8 aa, synthetic construct
  REGION 1..8: note = Synthetic Construct
ISSGGDNT

SEQ ID NO: 59 - protein, 8 aa, synthetic construct
  REGION 1..8: note = Synthetic Construct
IYPGDSDT

SEQ ID NO: 60 - protein, 8 aa, synthetic construct
  REGION 1..8: note = Synthetic Construct
INWNGGST

SEQ ID NO: 61 - protein, 7 aa, synthetic construct
  REGION 1..7: note = Synthetic Construct
AIYGNSY

SEQ ID NO: 62 - protein, 11 aa, synthetic construct
  REGION 1..11: note = Synthetic Construct
ARFDYGSSLDS

SEQ ID NO: 63 - protein, 11 aa, synthetic construct
  REGION 1..11: note = Synthetic Construct
ARFDYGSSLDC

SEQ ID NO: 64 - protein, 13 aa, synthetic construct
  REGION 1..13: note = Synthetic Construct
ARRGYRSSWYFDY

SEQ ID NO: 65 - protein, 11 aa, synthetic construct
  REGION 1..11: note = Synthetic Construct
AREGGELLMDY

SEQ ID NO: 66 - protein, 11 aa, synthetic construct
  REGION 1..11: note = Synthetic Construct
KSLLHSNGNTY

SEQ ID NO: 67 - protein, 6 aa, synthetic construct
  REGION 1..6: note = Synthetic Construct
QSISNN

SEQ ID NO: 68 - protein, 6 aa, synthetic construct
  REGION 1..6: note = Synthetic Construct
QSISNY

SEQ ID NO: 69 - protein, 6 aa, synthetic construct
  REGION 1..6: note = Synthetic Construct
QGIRND

SEQ ID NO: 70 - protein, 6 aa, synthetic construct
  REGION 1..6: note = Synthetic Construct
QSVSTY

SEQ ID NO: 71-75 - skipped (5 entries)

SEQ ID NO: 76 - protein, 9 aa, synthetic construct
  REGION 1..9: note = Synthetic Construct
MQGLEYPYT

SEQ ID NO: 77 - protein, 9 aa, synthetic construct
  REGION 1..9: note = Synthetic Construct
QQSKNWPRT

SEQ ID NO: 78 - protein, 9 aa, synthetic construct
  REGION 1..9: note = Synthetic Construct
QQSKSWPRT

SEQ ID NO: 79 - protein, 9 aa, synthetic construct
  REGION 1..9: note = Synthetic Construct
LQDYNYPLT

SEQ ID NO: 80 - protein, 9 aa, synthetic construct
  REGION 1..9: note = Synthetic Construct
QQRSNWPPT

SEQ ID NO: 81 - protein, 8 aa, synthetic construct
  REGION 1..8: note = Synthetic Construct
GFTFSHYS

SEQ ID NO: 82 - protein, 8 aa, synthetic construct
  REGION 1..8: note = Synthetic Construct
GFTFSWYP

SEQ ID NO: 83 - protein, 8 aa, synthetic construct
  REGION 1..8: note = Synthetic Construct
GFTFSDYE

SEQ ID NO: 84 - protein, 8 aa, synthetic construct
  REGION 1..8: note = Synthetic Construct
GFTFSYYD

SEQ ID NO: 85 - protein, 8 aa, synthetic construct
  REGION 1..8: note = Synthetic Construct
GFTFSHYQ

SEQ ID NO: 86 - protein, 8 aa, synthetic construct
  REGION 1..8: note = Synthetic Construct
GYTFTGYY

SEQ ID NO: 87 - protein, 8 aa, synthetic construct
  REGION 1..8: note = Synthetic Construct
GNTFTGYY

SEQ ID NO: 88 - protein, 8 aa, synthetic construct
  REGION 1..8: note = Synthetic Construct
GFTFSSYG

SEQ ID NO: 89 - protein, 8 aa, synthetic construct
  REGION 1..8: note = Synthetic Construct
GFTFSSYA

SEQ ID NO: 90 - protein, 8 aa, synthetic construct
  REGION 1..8: note = Synthetic Construct
GFTFSGYG

SEQ ID NO: 91 - protein, 8 aa, synthetic construct
  REGION 1..8: note = Synthetic Construct
GFTFSSFG

SEQ ID NO: 92 - protein, 8 aa, synthetic construct
  REGION 1..8: note = Synthetic Construct
GFTFNRFV

SEQ ID NO: 93 - protein, 8 aa, synthetic construct
  REGION 1..8: note = Synthetic Construct
GGSFSGYY

SEQ ID NO: 94 - protein, 8 aa, synthetic construct
  REGION 1..8: note = Synthetic Construct
GYTFTSYE

SEQ ID NO: 95 - protein, 8 aa, synthetic construct
  REGION 1..8: note = Synthetic Construct
GFTFSRYA

SEQ ID NO: 96 - protein, 7 aa, synthetic construct
  REGION 1..7: note = Synthetic Construct
IYPSGGT

SEQ ID NO: 97 - protein, 8 aa, synthetic construct
  REGION 1..8: note = Synthetic Construct
IYPSGGTT

SEQ ID NO: 98 - protein, 8 aa, synthetic construct
  REGION 1..8: note = Synthetic Construct
IWPSGGLT

SEQ ID NO: 99 - protein, 8 aa, synthetic construct
  REGION 1..8: note = Synthetic Construct
IYSSGGHT

SEQ ID NO: 100 - protein, 8 aa, synthetic construct
  REGION 1..8: note = Synthetic Construct
ISPSGGFT

SEQ ID NO: 101 - protein, 8 aa, synthetic construct
  REGION 1..8: note = Synthetic Construct
INPNSGGT

SEQ ID NO: 102 - protein, 8 aa, synthetic construct
  REGION 1..8: note = Synthetic Construct
IKPSTGDT

SEQ ID NO: 103 - protein, 8 aa, synthetic construct
  REGION 1..8: note = Synthetic Construct
IWYDGSNK

SEQ ID NO: 104 - protein, 8 aa, synthetic construct
  REGION 1..8: note = Synthetic Construct
ISGRGGSP

SEQ ID NO: 105 - protein, 8 aa, synthetic construct
  REGION 1..8: note = Synthetic Construct
IWSDGSNR

SEQ ID NO: 106 - protein, 8 aa, synthetic construct
  REGION 1..8: note = Synthetic Construct
IYYDGSNK

SEQ ID NO: 107 - protein, 8 aa, synthetic construct
  REGION 1..8: note = Synthetic Construct
ISGSGGST

SEQ ID NO: 108 - protein, 7 aa, synthetic construct
  REGION 1..7: note = Synthetic Construct
INHSGGT

SEQ ID NO: 109 - protein, 8 aa, synthetic construct
  REGION 1..8: note = Synthetic Construct
IYPRDGDT

SEQ ID NO: 110 - protein, 8 aa, synthetic construct
  REGION 1..8: note = Synthetic Construct
ISSGGDYI

SEQ ID NO: 111 - protein, 19 aa, synthetic construct
  REGION 1..19: note = Synthetic Construct
ARHWRGYSSSWYHPAYFDY

SEQ ID NO: 112 - protein, 19 aa, synthetic construct
  REGION 1..19: note = Synthetic Construct
ARSYYYDSSGYYSHDAFDI

SEQ ID NO: 113 - protein, 15 aa, synthetic construct
  REGION 1..15: note = Synthetic Construct
ARDSYYYDSSGALGY

SEQ ID NO: 114 - protein, 17 aa, synthetic construct
  REGION 1..17: note = Synthetic Construct
ARPGYSSGWYDGTYFDY

SEQ ID NO: 115 - protein, 12 aa, synthetic construct
  REGION 1..12: note = Synthetic Construct
TREPGRLWAFDI

SEQ ID NO: 116 - protein, 8 aa, synthetic construct
  REGION 1..8: note = Synthetic Construct
AVFGSGSS

SEQ ID NO: 117 - protein, 8 aa, synthetic construct
  REGION 1..8: note = Synthetic Construct
AVFGSGSS

SEQ ID NO: 118 - protein, 17 aa, synthetic construct
  REGION 1..17: note = Synthetic Construct
AREGGWYGGDYYYGMDV

SEQ ID NO: 119 - protein, 15 aa, synthetic construct
  REGION 1..15: note = Synthetic Construct
AKDGDGSGPPYYFDY

SEQ ID NO: 120 - protein, 24 aa, synthetic construct
  REGION 1..24: note = Synthetic Construct
ARDRGITMVRGLIIKYYYYYGLDV

SEQ ID NO: 121 - protein, 13 aa, synthetic construct
  REGION 1..13: note = Synthetic Construct
ARDDNWNDGDFDY

SEQ ID NO: 122 - protein, 19 aa, synthetic construct
  REGION 1..19: note = Synthetic Construct
AKDFTYYYGSGNYYNWFDP

SEQ ID NO: 123 - protein, 15 aa, synthetic construct
  REGION 1..15: note = Synthetic Construct
ARTSDYDYYYYGMDV

SEQ ID NO: 124 - protein, 8 aa, synthetic construct
  REGION 1..8: note = Synthetic Construct
ARHTPGAF

SEQ ID NO: 125 - protein, 17 aa, synthetic construct
  REGION 1..17: note = Synthetic Construct
TRVLFYYYGSSYVFFDY

SEQ ID NO: 126 - protein, 6 aa, synthetic construct
  REGION 1..6: note = Synthetic Construct
QSVSSY

SEQ ID NO: 127 - protein, 6 aa, synthetic construct
  REGION 1..6: note = Synthetic Construct
QSIDTY

SEQ ID NO: 128 - protein, 6 aa, synthetic construct
  REGION 1..6: note = Synthetic Construct
QSVSNW

SEQ ID NO: 129 - protein, 6 aa, synthetic construct
  REGION 1..6: note = Synthetic Construct
QSIDTW

SEQ ID NO: 130 - protein, 6 aa, synthetic construct
  REGION 1..6: note = Synthetic Construct
QDIRNW

SEQ ID NO: 131 - protein, 6 aa, synthetic construct
  REGION 1..6: note = Synthetic Construct
QGISNS

SEQ ID NO: 132 - protein, 6 aa, synthetic construct
  REGION 1..6: note = Synthetic Construct
QGISNY

SEQ ID NO: 133 - protein, 6 aa, synthetic construct
  REGION 1..6: note = Synthetic Construct
QGISSA

SEQ ID NO: 134 - protein, 6 aa, synthetic construct
  REGION 1..6: note = Synthetic Construct
QGISSW

SEQ ID NO: 135 - protein, 6 aa, synthetic construct
  REGION 1..6: note = Synthetic Construct
QSVSSY

SEQ ID NO: 136 - protein, 6 aa, synthetic construct
  REGION 1..6: note = Synthetic Construct
QGISSY

SEQ ID NO: 137 - protein, 6 aa, synthetic construct
  REGION 1..6: note = Synthetic Construct
QSISSW

SEQ ID NO: 138 - protein, 9 aa, synthetic construct
  REGION 1..9: note = Synthetic Construct
SGINLGRYR

SEQ ID NO: 139 - protein, 11 aa, synthetic construct
  REGION 1..11: note = Synthetic Construct
QSLVHSNGDTY

SEQ ID NO: 140 - protein, 6 aa, synthetic construct
  REGION 1..6: note = Synthetic Construct
QDISNF

SEQ ID NO: 141-152 - skipped (12 entries)

SEQ ID NO: 153 - protein, 7 aa, synthetic construct
  REGION 1..7: note = Synthetic Construct
YYSDSSK

SEQ ID NO: 154 - skipped

SEQ ID NO: 155 - protein, 9 aa, synthetic construct
  REGION 1..9: note = Synthetic Construct
QQRSNWPLT

SEQ ID NO: 156 - protein, 10 aa, synthetic construct
  REGION 1..10: note = Synthetic Construct
QQSYSSPGIT

SEQ ID NO: 157 - protein, 9 aa, synthetic construct
  REGION 1..9: note = Synthetic Construct
LQYVSYPLT

SEQ ID NO: 158 - protein, 9 aa, synthetic construct
  REGION 1..9: note = Synthetic Construct
QQYKTYPFT

SEQ ID NO: 159 - protein, 9 aa, synthetic construct
  REGION 1..9: note = Synthetic Construct
QQADSSPRT

SEQ ID NO: 160 - protein, 9 aa, synthetic construct
  REGION 1..9: note = Synthetic Construct
QQYKSYPYT

SEQ ID NO: 161 - protein, 9 aa, synthetic construct
  REGION 1..9: note = Synthetic Construct
QQYKTYPYT

SEQ ID NO: 162 - protein, 9 aa, synthetic construct
  REGION 1..9: note = Synthetic Construct
HQFNNYPFT

SEQ ID NO: 163 - protein, 9 aa, synthetic construct
  REGION 1..9: note = Synthetic Construct
QQYNSYPYT

SEQ ID NO: 164 - protein, 8 aa, synthetic construct
  REGION 1..8: note = Synthetic Construct
QQRSNWWT

SEQ ID NO: 165 - protein, 9 aa, synthetic construct
  REGION 1..9: note = Synthetic Construct
QQLNSYPRT

SEQ ID NO: 166 - protein, 9 aa, synthetic construct
  REGION 1..9: note = Synthetic Construct
QQYNSYSRT

SEQ ID NO: 167 - protein, 10 aa, synthetic construct
  REGION 1..10: note = Synthetic Construct
MIWHRSALFI

SEQ ID NO: 168 - protein, 9 aa, synthetic construct
  REGION 1..9: note = Synthetic Construct
SQSTHVPYT

SEQ ID NO: 169 - protein, 9 aa, synthetic construct
  REGION 1..9: note = Synthetic Construct
QQGHTLPYT

SEQ ID NO: 170 - protein, 113 aa, synthetic construct
  REGION 1..113: note = Synthetic Construct
QVQLQQSGPELVKPGASVKMSCKASGFTFTDSVISWVKQRTGQGLEWIGEIYPGSGSIYYNEKFKGKATLTADKSSNTAYMQLRSLTSEDSAVYFCAMRRSYWGQGTLVTVSA

SEQ ID NO: 171 - protein, 112 aa, synthetic construct
  REGION 1..112: note = Synthetic Construct
DVLMTQTPLSLPVSLGDQASISCRSSQSIVHSNGNTYLEWYLQKPGQSPKLLIYKVSNRFSGVPDRFSGSGSGTDFTLKISRVEAEDLGVYYCFQGSHVPLTFGAGTKLELK

SEQ ID NO: 172 - protein, 113 aa, synthetic construct
  REGION 1..113: note = Synthetic Construct
QIQLQQSGPELVKPGASVKMSCEASGFTFTDSVITWVKQRPGQGLEWIGEIYPGSGNFYYNEKFKGKATLTADKSSNTAYMQLRSLTSEDSAVYFCAMRRSSWGQGTLVTVSA

SEQ ID NO: 173 - protein, 112 aa, synthetic construct
  REGION 1..112: note = Synthetic Construct
DVLMTQTPLSLPVSLGDQASISCRSSQTIVHSNSKTYLEWYLQKPGQSPKLLIYKVSNRFSGVPDRFSGSGSGTDFTLKISRVEAEDLGVYYCFQGSHVPLTFGAGTKLELK

SEQ ID NO: 174 - protein, 125 aa, synthetic construct
  REGION 1..125: note = Synthetic Construct
QVQLQQSGGGLVQPGGSLRLSCAASGFTFSSYAMSWVRQAPGKGLEWVSAISGSGGSTYYADSVKGRFTVSRDNSKNTLYLQMNSLRAEDTAVYYCARLGYCSSTSCYLSAFDIWGQGTMVTVSS

SEQ ID NO: 175 - protein, 107 aa, synthetic construct
  REGION 1..107: note = Synthetic Construct
EIVLTQSPSTLSASVGDRVTITCRASQSISSWLAWYQQKPGKAPKLLIYDASSLESGVPSRFSGSGSGTEFTLTISSLQPDDFATYYCQQYNSYPLTFGGGTKVEIK

SEQ ID NO: 176 - protein, 120 aa, synthetic construct
  REGION 1..120: note = Synthetic Construct
QIQLVQSGAEVKKPGKSLKIACKGSGYSFSNYWIGWVRQMPGKGLEWMGIIYPGDSDTRYSPSFHGQVTISADKSISTAYLQWSSLKASDTAMYYCRVIINGTTSGFDYWGQGTLVIVSS

SEQ ID NO: 177 - protein, 107 aa, synthetic construct
  REGION 1..107: note = Synthetic Construct
ETTLTQSPATLSVSPGERATLSCRASQSVSSNLAWYQQKPGQAPRLLMYGASTRATGIPARFSGSGSGTEFTLTISSLQSEDFAVYYCQHYNNLPLTFGGGTKVDLK

SEQ ID NO: 178 - protein, 117 aa, synthetic construct
  REGION 1..117: note = Synthetic Construct
EVQLQQSGAELVKPGASVKLSCTASGFNIKDTYIHWVKQRPEQGLEWIGRIDPANGNTKYDPKFQGKATITADTSSNIVYVQFSSLTSEDTAVYYCGRSGGNYVGYWGQGTTLTVSS

SEQ ID NO: 179 - protein, 113 aa, synthetic construct
  REGION 1..113: note = Synthetic Construct
DIVMSQSPSSPTVSVGEKVTMTCKSSQSLLDSGNQKNYLAWYQQKPGQSPKLLIYWASTRKSGVPDRFTGSGSGTDFTLSISSVKAEDLAVYYCQQYYTYPWTFGGGTKLEIK

SEQ ID NO: 180 - protein, 117 aa, synthetic construct
  REGION 1..117: note = Synthetic Construct
EVQLQQSGAELVKPGASVKLSCTASGFNIKDTYMHWVKERPEQGLEWIGRIDPANGNTKYDPKFQGKATITADTSSNTAYLQLSSLTSEDTAVYYCGRSRGNYFDYWGQGTTLTVSS

SEQ ID NO: 181 - protein, 111 aa, synthetic construct
  REGION 1..111: note = Synthetic Construct
DIVMSQPPSSLAVSVGEKVTMTCKSSQSLKSNQKNYLAWYQQKPGQSPKLLIYWASTRESGVPDRFTGSGSGTDFTLTISSVKAEDLAVYYCQQYYTYPWTFGGGTKLEIK

SEQ ID NO: 182 - protein, 113 aa, synthetic construct
  REGION 1..113: note = Synthetic Construct
QVQLVQSGAEVKKPGTSVKVSCKASGYTFTTYYMHWVRQAPGQGLEWMGLINPSAGNTRNAQKFQGRVTMTRDTSTNTVYMELSSLRSEDTAVYYCARELDIWGQGTKVTVSS

SEQ ID NO: 183 - protein, 107 aa, synthetic construct
  REGION 1..107: note = Synthetic Construct
AIQMTQSPSSLSASVGDRVTITCRASQDIRNDLGWYQQKPGKAPKLLIYAASSLQSGVPSRFSGNGSGTDFTLTINSLQPEDFATYYCLQDFNFPFTFGPGTTVDIN

SEQ ID NO: 184 - protein, 120 aa, synthetic construct
  REGION 1..120: note = Synthetic Construct
QVQLVESGGGVVQSGRSLRLSCAASGFTFSSYGMHWVRQAPGKGLEWVAVIWYDGSNKYYADSVKDRFTISRDNSKKTVYLQMNSLRAEDTAVYYCAREGMVRGALFDYWGQGTLVTVSS

SEQ ID NO: 185 - protein, 108 aa, synthetic construct
  REGION 1..108: note = Synthetic Construct
EIVMTQSPATLSLSPGERATLSCRASQSVSSSYLSWYQQKPGQAPRLLIYGASTRATGIPARFSGSGSGPDLTLTISSLQPEDFAVYYCQQDYNLPYTFGQGTKLEIK

SEQ ID NO: 186 - protein, 119 aa, synthetic construct
  REGION 1..119: note = Synthetic Construct
EVQLVQSGAEVKKPGESLKISCKGSGYSFTSYWIGWVRQMPGKGLEWMGVIYPGDSDTRYSPSFQGQVTMSADKSISTAYLQWSSLKASDSAMYYCARQLRDYYGMDVWGQGTTVTVSS

SEQ ID NO: 187 - protein, 108 aa, synthetic construct
  REGION 1..108: note = Synthetic Construct
EIVMTQSPATLSLSPGERATLSCRASQTISSNYFSWYQQKPGQAPRLLIYGASTRATGIPARFSGSGSETDFTLTISSLQPEDFAVYYCQQDYNLPRTFGQGTKVEIK

SEQ ID NO: 188 - protein, 119 aa, synthetic construct
  REGION 1..119: note = Synthetic Construct
EVQLVQSGAEVKKPGESLKISCKGSGYSFTSYWIGWVRQMPGKGLEWMGIIYPGDSDTRYSPSFQGQVTISADKSISTAYLHWSSLKASDTAMYYCARQLRDYYSMDVWGQGTTVTVSS

SEQ ID NO: 189 - protein, 108 aa, synthetic construct
  REGION 1..108: note = Synthetic Construct
EIVMTQSPATLSLSPGERATLSCRASQSVSSSYLSWYQQKPGQAPRLLIYGASTRATGIAARFSGSGSGTDFTLTISSLQPEDFAVYYCQQDYNLPRTFGQGTKVEIK

SEQ ID NO: 190 - protein, 114 aa, synthetic construct
  REGION 1..114: note = Synthetic Construct
EVQLQQSGPELVKPGASVKMSCKASGYTFTSYNIHWVKQKPGQGLEWIGYINPYNDGTKYSEKFKGKATLTSDRSSSTAYMEVSSLTSEDSAVYYCAIYGNSYWGQGSTLTVSS

SEQ ID NO: 191 - protein, 112 aa, synthetic construct
  REGION 1..112: note = Synthetic Construct
DIVMTQAAPSIPVTPGESVSISCRSSKSLLHSNGNTYLYWFLQRPGQSPQRLIYYMSNLDSGVPDRFSGRGSGTDFTLRISRVEAEDVGVYYCMQGLEYPYTFGGGTKLEIK

SEQ ID NO: 192 - protein, 118 aa, synthetic construct
  REGION 1..118: note = Synthetic Construct
DVMLVESGGDLVKPGGSLKLSCAASGFTFSSYTMSWVRQTPEKRLEWVASISSGGGNTYYPDSVKGRFTISRDNAKNNLYLQMSSLRSEDTALYYCARFDYGSSLDSWGQGTTLTVSS

SEQ ID NO: 193 - protein, 107 aa, synthetic construct
  REGION 1..107: note = Synthetic Construct
DIVLTQSPATLSVTPGDSVSLSCRASQSISNNLHWYQQKSHESPRLLIKYASQSISGIPSRFSGSGSGTDFTLSINSVETEDFGMYFCQQSKNWPRTFGGGTKLEIK

SEQ ID NO: 194 - protein, 118 aa, synthetic construct
  REGION 1..118: note = Synthetic Construct
EVMLVESGGGLVKPGGSLKLSCAASGFTFSSYTMSWVRQTPEKRLEWVATISSGGDNTYYPDSVKGRFTISRDNAKNNLYLQMSSLRSEDTALYYCARFDYGSSLDCWGQGTTLTVSS

SEQ ID NO: 195 - protein, 107 aa, synthetic construct
  REGION 1..107: note = Synthetic Construct
DIVLTQSPATLSVTPGDSVSLSCRASQSISNYLHWYQQKSHESPRLLIKYASQSISGIPSRFSGSGSGTDFTLSINSVETEDFGMYFCQQSKSWPRTFGGGTELEIK

SEQ ID NO: 196 - protein, 120 aa, synthetic construct
  REGION 1..120: note = Synthetic Construct
EVQLVQSGAEVKKPGESLKISCKGSGYSFTSYWIGWVRQMPGKGLEWMGIIYPGDSDTRYSPSFQGQVTISADKSISTAYLQWSSLKASDTAMYYCARRGYRSSWYFDYWGQGTLVTVSS

SEQ ID NO: 197 - protein, 107 aa, synthetic construct
  REGION 1..107: note = Synthetic Construct
AIQMTQSPSSLSASVGDRVTITCRASQGIRNDLGWYQQKPGKAPKLLIYAASSLQSGVPSRFSGSGSGTDFTFTISSLQPEDFATYYCLQDYNYPLTFGGGTKVEIK

SEQ ID NO: 198 - protein, 118 aa, synthetic construct
  REGION 1..118: note = Synthetic Construct
EVQLVESGGGVVRPGGSLRLSCAASGFTFDDYGMSWVRQAPGKGLEWVSGINWNGGSTGYADSVKGRFTISRDNAKNSLYLQMNSLRAEDTALYHCAREGGELLMDYWGQGTLVTVSS

SEQ ID NO: 199 - protein, 105 aa, synthetic construct
  REGION 1..105: note = Synthetic Construct
EIVLTQSPATLSLSPGERATLSCRASQSVSTYLAWYQQKPGQAPRLLIYDNRATGIPPRFSGSGSGTDFTLTISSLEPEDFAVYYCQQRSNWPPTFGGGTTVEIK

SEQ ID NO: 200 - protein, 125 aa, synthetic construct
  REGION 1..125: note = Synthetic Construct
EVQLLESGGGLVQPGGSLRLSCAASGFTFSHYSMVWVRQAPGKGLEWVSYIYPSGGTSYADSVKGRFTISRDNSKNTLYLQMNSLRAEDTAVYYCARHWRGYSSSWYHPAYFDYWGQGTLVTVSS

SEQ ID NO: 201 - protein, 105 aa, synthetic construct
  REGION 1..105: note = Synthetic Construct
DIQMTQSPATLSLSPGERATLSCRASQSVSSYLAWYQQKPGQAPRLLIYDNRATGIPARFSGSGSGTDFTLTISSLEPEDFAVYYCQQRSNWPLTFGGGTKVEIK

SEQ ID NO: 202 - protein, 126 aa, synthetic construct
  REGION 1..126: note = Synthetic Construct
EVQLLESGGGLVQPGGSLRLSCAASGFTFSWYPMMWVRQAPGKGLEWVSSIYPSGGTTTYADSVKGRFTISRDNSKNTLYLQMNSLRAEDTAVYYCARSYYYDSSGYYSHDAFDIWGQGTMVTVSS

SEQ ID NO: 203 - protein, 108 aa, synthetic construct
  REGION 1..108: note = Synthetic Construct
DIQMTQSPSSLSASVGDRVAITCRASQSIDTYLNWYQQKPGKAPKLLIYAASKLEDGVPSRFSGSGTGTDFTLTIRSLQPEDFASYFCQQSYSSPGITFGPGTKVEIK

SEQ ID NO: 204 - protein, 122 aa, synthetic construct
  REGION 1..122: note = Synthetic Construct
EVQLLESGGGLVQPGGSLRLSCAASGFTFSDYEMHWVRQAPGKGLEWVSSIWPSGGLTKYADPVKGRFTISRDNSKNTLYLQMNSLRAEDTAVYYCARDSYYYDSSGALGYWGQGTLVTVSS

SEQ ID NO: 205 - protein, 107 aa, synthetic construct
  REGION 1..107: note = Synthetic Construct
DIQMTQSPSTLSASVGDRVTITCRASQSVSNWLAWYQQKPGKAPKLLIYKASSLESGVPSRFSGSGSGTEFTLTISSLQPDDFATYYCLQYVSYPLTFGGGTKVDIK

SEQ ID NO: 206 - protein, 124 aa, synthetic construct
  REGION 1..124: note = Synthetic Construct
EVQLLESGGGLVQPGGSLRLSCAASGFTFSYYDMYWVRQAPGKGLEWVSRIYSSGGHTWYADSVKGRFTISRDNSKNTLYLQMNSLRAEDTAVYYCARPGYSSGWYDGTYFDYWGQGTLVTVSS

SEQ ID NO: 207 - protein, 107 aa, synthetic construct
  REGION 1..107: note = Synthetic Construct
DIQMTQSPSTLSASVGDRVTITCRASQSIDTWLAWYRQKPGKAPNVVIHSASTLQSGVPARFSGSGFGTEWTLTITNLQPDDFATYYCQQYKTYPFTFGQGTKLEIK

SEQ ID NO: 208 - protein, 119 aa, synthetic construct
  REGION 1..119: note = Synthetic Construct
EVQLLESGGGLVQPGGSLRLSCAASGFTFSHYQMEWVRQAPGKGLEWVSSISPSGGFTSYADSVKGRFTISRDNSKNTLYLQMNSLRAEDTAVYYCTREPGRLWAFDIWGQGTMVTVSS

SEQ ID NO: 209 - protein, 107 aa, synthetic construct
  REGION 1..107: note = Synthetic Construct
DIQMTQSPSFVSASVGDRVTITCRASQDIRNWLAWYQQESGKAPRLLISAASSRHSGVSSRFSGSGSGTDFTLTITSLQPEDSATYFCQQADSSPRTFGQGTKVEIK

SEQ ID NO: 210 - protein, 115 aa, synthetic construct
  REGION 1..115: note = Synthetic Construct
QVQLVQSGAEVKKPGASVKVSCKASGYTFTGYYMHWVRQAPGQGLEWMGWINPNSGGTNYAQKFQGRVTMTRDTSINTAYMELSRLRSDDTAVYYCAVFGSGSSWGQGTLVTVSS

SEQ ID NO: 211 - protein, 107 aa, synthetic construct
  REGION 1..107: note = Synthetic Construct
DIQMTQSPSSLSASVGDRVTITCRASQGISNSLAWFQQKPGKAPKSLIYAASSLQSGVPSKFSGSGSGTDFTLTISSLQPEDFATYYCQQYKSYPYTFGQGTKLEIK

SEQ ID NO: 212 - protein, 115 aa, synthetic construct
  REGION 1..115: note = Synthetic Construct
QVQLVQSGAEVKKPGASVKVSCKASGNTFTGYYIHWVRQAPGQGLEWMGWIKPSTGDTNYAQNFLDRVTMTRDTSISTAYMELSRLRSDDTAVYYCAVFGSGSSWGQGTLVTVSS

SEQ ID NO: 213 - protein, 107 aa, synthetic construct
  REGION 1..107: note = Synthetic Construct
DIHMTQSPSSLSAFVGDRVTITCRASQGISNYLAWFQQKPGKAPKSLIYAASSLQSGVPSKFSGSGSGTDFTLTINNLQPEDFATYYCQQYKTYPYTFGQGTKLEIK

SEQ ID NO: 214 - protein, 124 aa, synthetic construct
  REGION 1..124: note = Synthetic Construct
QVQLVESGGGVVQPGRSLRLSCAASGFTFSSYGMHWVRQAPGKGLEWVAVIWYDGSNKYYADSVKGRFTISRDNSKNTLYLQMNSLRAEDAAVYYCAREGGWYGGDYYYGMDVWGQGTTVTVSS

SEQ ID NO: 215 - protein, 105 aa, synthetic construct
  REGION 1..105: note = Synthetic Construct
AIQLTQSPSSLSASVGDRVTITCRASQGISSAWYQQKPGKAPKLLIYDASSLESGVPSRFSGSGSGTDFTLTISSLQPEDFATYYCHQFNNYPFTFGPGTKVDIK

SEQ ID NO: 216 - protein, 122 aa, synthetic construct
  REGION 1..122: note = Synthetic Construct
EVQLLESGGGLVQPGGSLRLSCVASGFTFSSYAMSWVRQAPGKGLEWVSGISGRGGSPNYADSVKGRFTISRDNSKNTLYLQMNSLRAEDTAVYYCAKDGDGSGPPYYFDYWGQGTLVTVSS

SEQ ID NO: 217 - protein, 107 aa, synthetic construct
  REGION 1..107: note = Synthetic Construct
DIQMTQSPSSLSASVGDRVTITCRASQGISSWLAWYQQKPEKAPKSLIYAASSLQSGVPSRFSGSGSGTDFTLTISSLQPEDFATYYCQQYNSYPYTFGQGTKLEIK

SEQ ID NO: 218 - protein, 131 aa, synthetic construct
  REGION 1..131: note = Synthetic Construct
QVQLMESGGGVVQPGRSLRLSCAASGFTFSGYGMHWVRQAPGKGLEWVAVIWSDGSNRYYTDSVKGRFTISRDNSKNTLSLQMNSLRAEDTAVYYCARDRGITMVRGLIIKYYYYYGLDVWGQGTSVTVSS

SEQ ID NO: 219 - protein, 104 aa, synthetic construct
  REGION 1..104: note = Synthetic Construct
EIVLTQSPATLSLSPGERATLSCRASQSVSSYLAWYQQKPGQAPRLLIYDNRATGIPARFSGSGSGTDFTLTISSLEPEDFAVYYCQQRSNWWTFGQGTKVEIK

SEQ ID NO: 220 - protein, 120 aa, synthetic construct
  REGION 1..120: note = Synthetic Construct
QVQLVESGGGVVQPGRSLRLSCAASGFTFSSFGMHWVRQAPGKGLEWVAVIYYDGSNKYYADSVKGRFTISRDNSKNTLYLQMNSLRAEDTAVYYCARDDNWNDGDFDYWGQGTLVTVSS

SEQ ID NO: 221 - protein, 107 aa, synthetic construct
  REGION 1..107: note = Synthetic Construct
DIQLTQSPSFLSASVGDRVTITCRASQGISSYLAWYQQKPGKAPKLLIYAASTLQSGVPSRFSGSGSGTEFTLTISSLQPEDFATYYCQQLNSYPRTFGQGTKVEIK

SEQ ID NO: 222 - protein, 126 aa, synthetic construct
  REGION 1..126: note = Synthetic Construct
EVQLLESGGGLVQPGESLRLSCAASGFTFNRFVMSWVRQAPGKGLEWVSTISGSGGSTYYADSVKGRFTISRDNSKNTLYLQMNSLRAEDTAVYYCAKDFTYYYGSGNYYNWFDPRGQGTLVTVSS

SEQ ID NO: 223 - protein, 107 aa, synthetic construct
  REGION 1..107: note = Synthetic Construct
DIQMTQSPSTLSTSVGDRVTITCRASQSISSWLAWYQQKPGKAPKLLIYKASSLESGVPSRFSGSGSGTEFTLTISSLQPDDFATYYCQQYNSYSRTFGQGTKVEIK

SEQ ID NO: 224 - protein, 121 aa, synthetic construct
  REGION 1..121: note = Synthetic Construct
QVQLQQWGAGLLKPSETLSLTCAVYGGSFSGYYWSWIRQPPGKGLEWIGEINHSGGTNYNPSLKSRVTISVDTSKNHFSLKLSSVTAADTAVYYCARTSDYDYYYYGMDVWGQGTTVTVSS

SEQ ID NO: 225 - protein, 114 aa, synthetic construct
  REGION 1..114: note = Synthetic Construct
QPVLTQPTSLSDGASARLTCTLRSGINLGRYRIFWYQQKPESPPRYLLSYYSDSSKHQGSGVPSRFSGSKDASSNAGILVISGLQSEDEADYYCMIWHRSALFIFGSGTKVTVL

SEQ ID NO: 226 - protein, 115 aa, synthetic construct
  REGION 1..115: note = Synthetic Construct
QVQLQQSGPELVKPGASVKLSCKASGYTFTSYEINWLKQRPGQGLEWIGLIYPRDGDTKYNEKFKGKATLTADTSSSTAYMELHSLTSEDSAVYFCARHTPGAFWGQGTLVTVSA

SEQ ID NO: 227 - protein, 112 aa, synthetic construct
  REGION 1..112: note = Synthetic Construct
DVVMTQTPLSLPVSLGDQASISCRSSQSLVHSNGDTYLHWYLQKPGQSPKLLIYKVSNRFSGVPDRFSGSGSGTDFTLKISRVEAEDLEIYFCSQSTHVPYTFGGGTKLEIK

SEQ ID NO: 228 - protein, 124 aa, synthetic construct
  REGION 1..124: note = Synthetic Construct
DVKLVESGEGLVKPGGSLKLSCAASGFTFSRYAMSWVRQTPEKRLEWVAYISSGGDYIHYGETVKGRFTISRDNARNTLYLQMSSLKSEDTAMYYCTRVLFYYYGSSYVFFDYWGQGTTLTVSS

SEQ ID NO: 229 - protein, 107 aa, synthetic construct
  REGION 1..107: note = Synthetic Construct
DIQMTQTTSSLSVSLGDRVTISCRASQDISNFLNWYQQKPDGTVNLLIYYTSKLHSGVPSRFSGGGSGRDYSLTINNLEQEDIASYFCQQGHTLPYTFGGGTKLEIK

SEQ ID NO: 230 - DNA, 339 bp, synthetic construct
  misc_feature 1..339: note = Synthetic Construct
  source 1..339: mol_type = other DNA
caggtgcagctgcagcagagcggtcccgagctggtgaaacctggcgcatcagtcaaaatgagctgcaaggcctccggcttcacttttaccgactcagtgatcagctgggtcaagcagcgaaccggtcagggactggagtggatcggagaaatctaccctggatctgggagtatctactataacgagaagttcaaagggaaggcaacactgactgccgacaaaagctccaatacagcctatatgcagctgcgatccctgacttctgaagatagcgccgtgtacttttgcgcaatgcggaggtcctattggggtcagggcaccctggtgacagtctctgct

SEQ ID NO: 231 - DNA, 336 bp, synthetic construct
  misc_feature 1..336: note = Synthetic Construct
  source 1..336: mol_type = other DNA
gacgtgctgatgacccagacacccctgagtctgcctgtctcactgggagatcaggcttctatcagttgccgaagctcccagagcatcgtgcattccaacggaaatacctacctggagtggtatctgcagaagccagggcagtcccccaagctgctgatctacaaagtgtctaaccggttcagtggcgtcccagacaggttttcaggtagcggctccggaactgatttcaccctgaaaatttcccgggtggaggcagaagacctgggtgtctactattgcttccagggcagccatgtgcccctgacttttggggccggtaccaagctggagctgaaa

SEQ ID NO: 232 - DNA, 339 bp, synthetic construct
  misc_feature 1..339: note = Synthetic Construct
  source 1..339: mol_type = other DNA
cagatccagctgcagcagtccggtcccgagctggtgaaacctggcgcatctgtcaagatgagttgcgaagcctcaggcttcacttttaccgactccgtgattacctgggtcaaacagcgcccaggccagggactggagtggatcggagaaatctaccccggatctgggaacttctactataatgagaagtttaaagggaaggcaacactgactgccgacaagagctccaacaccgcctacatgcagctgcgatcactgacaagcgaagatagcgccgtgtacttctgcgcaatgcggaggtctagttggggtcagggcaccctggtgacagtctctgct

SEQ ID NO: 233 - DNA, 336 bp, synthetic construct
  misc_feature 1..336: note = Synthetic Construct
  source 1..336: mol_type = other DNA
gacgtgctgatgacccagacacccctgtctctgcctgtcagtctgggagatcaggcttctatcagttgccgaagctcccagaccatcgtgcattcaaacagcaagacatacctggagtggtatctgcagaaaccaggccagtcccccaagctgctgatctacaaagtgtcaaatcggttctctggagtcccagacaggttttccggttctggcagtggaactgatttcaccctgaagatttctcgggtggaggcagaagacctgggtgtctactattgcttccaggggagccatgtgcccctgacttttggggccggtaccaagctggagctgaaa

SEQ ID NO: 234 - DNA, 375 bp, synthetic construct
  misc_feature 1..375: note = Synthetic Construct
  source 1..375: mol_type = other DNA
caggtgcagctgcagcagtcggggggaggcttggtacagcctggggggtccctgagactctcctgtgcagcctctggattcacctttagcagctatgccatgagctgggtccgccaggctccagggaaggggctggagtgggtctcagctattagtggtagtggtggtagcacatactacgcagactccgtgaagggccggttcaccgtctccagagacaattccaagaacacgctgtatctgcaaatgaacagcctgagagccgaggacacggccgtatattactgtgcgaggctaggatattgtagtagtaccagctgctatttgtctgcttttgatatctggggccaagggacaatggtcaccgtctcttca

SEQ ID NO: 235 - DNA, 321 bp, synthetic construct
  misc_feature 1..321: note = Synthetic Construct
  source 1..321: mol_type = other DNA
gaaattgtgttgacacagtctccttccaccctgtctgcatctgtaggagacagagtcaccatcacttgccgggccagtcagagtattagtagctggttggcctggtatcagcagaaaccagggaaagcccctaagctcctgatctatgatgcctccagtttggaaagtggggtcccatcaaggttcagcggcagtggatctgggacagaattcactctcaccatcagcagcctgcagcctgatgattttgcaacttattactgccaacagtataatagttacccgctcactttcggcggagggaccaaggtggagatcaaa

SEQ ID NO: 236 - DNA, 366 bp, synthetic construct
  misc_feature 1..366: note = Synthetic Construct
  source 1..366: mol_type = other DNA
cagatccagctggtgcagtctggcgccgaagtgaagaagcctggcaagagcctgaagatcgcctgcaagggctccggctacagcttcagcaactactggatcggctgggtgcgccagatgcctggaaaaggactggaatggatgggcattatctaccctggcgacagcgacacccggtacagccccagcttccacggccaggtgacaatcagcgccgacaagagcatctccaccgcctacctgcagtggtcctccctgaaggccagcgacaccgccatgtactattgtgccagaggcgtgatcatcaacggcaccaccagcggcttcgactattggggacagggcaccctggtgatcgtgtcctcc

SEQ ID NO: 237 - DNA, 321 bp, synthetic construct
  misc_feature 1..321: note = Synthetic Construct
  source 1..321: mol_type = other DNA
gagacaaccctgacccagagccccgccaccctgtccgtgtctccaggcgagagagccaccctgagctgcagagccagccagagcgtgtccagcaacctggcctggtatcagcagaagcccggccaggcccccagactgctgatgtacggcgccagcaccagagccaccggcatccctgccagattcagcggcagcggctccggcaccgagttcaccctgaccatcagcagcctgcagagcgaggacttcgccgtgtactactgccagcactacaacaacctgcccctgaccttcggcggaggcaccaaggtggacctgaag

SEQ ID NO: 238 - DNA, 351 bp, synthetic construct
  misc_feature 1..351: note = Synthetic Construct
  source 1..351: mol_type = other DNA
gaagtccaactccaacagtctggggcagaacttgtcaaacctggggcttcagtaaaattgagttgcacagcaagtggctttaacatcaaagacacatatattcattgggtgaagcaacgaccagaacaaggcttggagtggatcggtaggattgaccctgcaaacgggaatacaaaatatgaccctaaattccagggaaaggctacaataacagcagacaccagcagtaacattgtctatgtgcaatttagctctcttacctctgaggacactgctgtctattattgcggacgtagtggcgggaattatgtgggttattggggccaggggacaacactcaccgtatcctct

SEQ ID NO: 239 - DNA, 339 bp, synthetic construct
  misc_feature 1..339: note = Synthetic Construct
  source 1..339: mol_type = other DNA
gatatagtaatgtcccagtctccttcatcacctactgtgtcagttggagaaaaagtcaccatgacctgtaagtcctcacagtccctcttggacagcgggaatcagaaaaattatctcgcatggtatcagcaaaagccagggcagtcccctaagctgttgatctattgggcaagtacaaggaaaagtggcgtgcctgatagattcacagggagcggcagcgggacagacttcactttgagcatctcttcagtaaaagccgaagacctggcagtgtactactgtcagcaatattatacctacccttggacttttggtggcgggaccaaactggaaataaaa

SEQ ID NO: 240 - DNA, 351 bp, synthetic construct
  misc_feature 1..351: note = Synthetic Construct
  source 1..351: mol_type = other DNA
gaggttcaacttcagcaatcaggggctgagcttgtaaaacctggagcctctgtaaaactctcttgtaccgcctccgggttcaacataaaagatacatatatgcactgggtaaaggagcggcccgaacagggactcgaatggatcgggaggattgacccagctaacggaaataccaagtatgatccaaaatttcaggggaaagctacaataaccgccgatacttctagtaatacagcatatcttcagctcagcagcttgacaagcgaagataccgcagtttactactgcggtcgatcccgagggaattattttgactactggggccagggtactactctcacagtaagtagc

SEQ ID NO: 241 - DNA, 339 bp, synthetic construct
  misc_feature 1..339: note = Synthetic Construct
  source 1..339: mol_type = other DNA
gacatagtaatgagccagccacctagttcacttgccgtaagtgtgggtgaaaaggtgactatgacctgtaaaagtagtcagagcctcctttactcatcaaatcagaagaattacttggcctggtatcaacagaaacctggacaaagccccaaactcctcatatactgggcctctacccgagagtccggcgtaccagatcggtttaccggttctggatcaggtacagactttacacttaccatctcttcagtgaaggctgaggacttggccgtgtattattgtcaacaatattatacatatccttggacttttggcggagggacaaagctcgaaataaag

SEQ ID NO: 242 - DNA, 339 bp, synthetic construct
  misc_feature 1..339: note = Synthetic Construct
  source 1..339: mol_type = other DNA
caggtgcagctggtgcagtctggcgccgaagtgaagaaacccggcacctccgtgaaggtgtcctgcaaggcttccggctacacctttaccacctactacatgcactgggtgcgacaggcccctggacagggcctggaatggatgggcctgatcaacccttccgccggcaacaccagaaacgcccagaaattccagggcagagtgaccatgacccgggacacctccaccaacaccgtgtacatggaactgtcctccctgcggagcgaggacaccgccgtgtactactgtgccagagagctggacatctggggccagggcaccaaagtgaccgtgtcctct

SEQ ID NO: 243 - DNA, 321 bp, synthetic construct
  misc_feature 1..321: note = Synthetic Construct
  source 1..321: mol_type = other DNA
gccatccagatgacccagtcccccagctccctgtctgcctctgtgggcgacagagtgaccatcacctgtcgggcctctcaggacatccggaacgacctgggctggtatcagcagaagcctggcaaggcccccaagctgctgatctacgccgcttccagtctccagtccggcgtgccctccagattctccggcaatggctctggcaccgacttcaccctgaccatcaactccctccagcccgaggacttcgccacctactactgtctccaagacttcaacttccccttcaccttcggccctggcaccaccgtggacatcaac

SEQ ID NO: 244 - DNA, 360 bp, synthetic construct
  misc_feature 1..360: note = Synthetic Construct
  source 1..360: mol_type = other DNA
caggtgcagctggtggagtctgggggaggcgtggtccagtctgggaggtccctgagactctcctgtgcagcgtctggattcaccttcagtagttatggcatgcactgggtccgccaggctccaggcaaggggctggagtgggtggcagttatatggtatgatggaagtaataaatactatgcagactccgtgaaggaccgattcaccatctccagagacaattccaagaaaacggtgtatctgcaaatgaacagtctgagagccgaggacacggctgtttattactgtgcgagagaagggatggttcggggagccctctttgactactggggtcagggaaccctggtcaccgtctcctca

SEQ ID NO: 245 - DNA, 324 bp, synthetic construct
  misc_feature 1..324: note = Synthetic Construct
  source 1..324: mol_type = other DNA
gaaattgtaatgacacagtctccagccaccctgtctttgtctccaggggaaagagccaccctctcctgcagggccagtcagagtgttagcagcagctacttatcctggtaccaacagaaacctgggcaggctcccaggctcctcatctatggtgcatccaccagggccactggcatcccagccaggttcagtggcagtgggtctgggccagacctcactctcaccatcagcagcctgcagcctgaagattttgcagtttattactgtcagcaggattataacttaccgtacacttttggccaggggaccaagctggagatcaaa

SEQ ID NO: 246 - DNA, 357 bp, synthetic construct
  misc_feature 1..357: note = Synthetic Construct
  source 1..357: mol_type = other DNA
gaggtgcagctggtgcagtctggagcagaggtgaaaaagcccggggagtctctgaagatctcctgtaagggttctggatacagttttactagttactggatcggctgggtgcgccagatgcccgggaaaggcctggagtggatgggagtcatctatcctggtgactctgataccagatatagcccgtccttccaaggccaggtcaccatgtcagccgacaagtccatcagtaccgcctacctgcagtggagcagcctgaaggcctcggacagcgccatgtattactgtgcgagacagctacgagactactacggtatggacgtctggggccaagggaccacggtcaccgtctcctca

SEQ ID NO: 247 - DNA, 324 bp, synthetic construct
  misc_feature 1..324: note = Synthetic Construct
  source 1..324: mol_type = other DNA
gaaattgtaatgacacagtctccagccaccctgtctttgtctccaggggaaagagccaccctctcctgcagggccagtcagactatcagcagcaactacttttcctggtaccagcagaaacctgggcaggctcccaggctcctcatctatggtgcatccaccagggccactggcattccagccaggttcagtggcagtgggtctgagacagacttcactctcaccatcagcagcctgcagcctgaagattttgcagtttattactgtcagcaggattataacttacctcggacgttcggccaagggaccaaggtggaaatcaaa

SEQ ID NO: 248 - DNA, 357 bp, synthetic construct
  misc_feature 1..357: note = Synthetic Construct
  source 1..357: mol_type = other DNA
gaggtgcagctggtgcagtctggagcagaggtgaaaaagcccggggagtctctgaagatctcctgtaagggttctggatacagctttaccagctactggatcggctgggtgcgccagatgcccgggaaaggcctggagtggatggggatcatctatcctggtgactctgataccagatacagcccgtccttccaaggccaggtcaccatctcagccgacaagtccatcagcaccgcctacctgcactggagcagcctgaaggcctcggacaccgccatgtattactgtgcgagacagctacgagactactacagtatggacgtctggggccaagggaccacggtcaccgtctcctca

SEQ ID NO: 249 - DNA, 324 bp, synthetic construct
  misc_feature 1..324: note = Synthetic Construct
  source 1..324: mol_type = other DNA
gaaattgtaatgacacagtctccagccaccctgtctttgtctccaggggaaagagccaccctctcctgcagggccagtcagagtgttagcagcagctacttatcctggtaccagcagaaacctgggcaggctcccaggctcctcatctatggtgcatccaccagggccactggcattgcagccaggttcagtggcagtgggtctgggacagacttcactctcaccatcagcagcctgcagcctgaagattttgcagtttattactgtcagcaggattataacttacctcggacgttcggccaagggaccaaggtggaaatcaaa

SEQ ID NO: 250 - DNA, 342 bp, synthetic construct
  misc_feature 1..342: note = Synthetic Construct
  source 1..342: mol_type = other DNA
gaggtgcagctgcagcagagcggccctgagctggtgaaacctggcgccagcgtgaagatgagctgcaaggccagcggctacaccttcaccagctacaacatccactgggtgaaacagaagcccggccagggcctggaatggattggctacatcaacccctacaacgacggcaccaagtacagcgagaagttcaagggcaaggccaccctgaccagcgacagaagcagcagcaccgcctacatggaagtgtccagcctgacctccgaggacagcgccgtgtactactgcgccatctacggcaacagctactggggccagggcagcaccctgaccgtgtccagc

SEQ ID NO: 251 - DNA, 336 bp, synthetic construct
  misc_feature 1..336: note = Synthetic Construct
  source 1..336: mol_type = other DNA
gacatcgtgatgacccaggctgcccccagcatccccgtgacacctggcgagtccgtgtccatcagctgcagaagcagcaagagcctgctgcacagcaacggcaatacctacctgtactggttcctgcagcggcctggccagtccccccagcggctgatctactacatgagcaacctggacagcggcgtgcccgaccggtttagcggcagaggcagcggcacagactttaccctgcggatcagccgggtggaagccgaggacgtgggcgtgtactattgcatgcagggcctggaatacccctacacctttggaggcggcaccaagctggaaatcaag

SEQ ID NO: 252 - DNA, 354 bp, synthetic construct
  misc_feature 1..354: note = Synthetic Construct
  source 1..354: mol_type = other DNA
gacgtgatgctggtcgagagcggcggagatctggtcaaacccgggggttctctgaagctgagttgtgccgcttcaggcttcactttttctagttacaccatgagctgggtgcgacagaccccagagaagcggctggaatgggtcgctagcatctcaagcggcggagggaacacctactatcccgactctgtgaaaggcagattcacaattagtcgcgataatgcaaagaacaatctgtacctgcagatgtcctctctgaggtccgaagatactgccctgtactattgtgctagatttgactatggaagttcactggattcttggggacaggggaccacactgacagtgagctcc

SEQ ID NO: 253 - DNA, 321 bp, synthetic construct
  misc_feature 1..321: note = Synthetic Construct
  source 1..321: mol_type = other DNA
gacatcgtcctgacccagagtcctgccaccctgtctgtgacaccaggcgattctgtcagtctgtcatgtagagctagccagtccatctctaacaatctgcactggtaccagcagaagtcacatgaaagccccagactgctgatcaagtatgccagtcagtcaatcagcggtattccttcccgcttctccggctctggaagtgggacagactttactctgtccatcaactctgtggagacagaagatttcggcatgtatttttgtcagcagagcaagaattggcccaggacatttggcggagggactaagctggagatcaag

SEQ ID NO: 254 - DNA, 354 bp, synthetic construct
  misc_feature 1..354: note = Synthetic Construct
  source 1..354: mol_type = other DNA
gaagtgatgctggtcgaaagtggaggaggactggtgaaaccaggtggaagcctgaagctgtcctgtgccgcttctggcttcactttttcaagctataccatgagctgggtgcgacagacacctgagaagcggctggaatgggtcgctacaatctcctctggaggggacaacacttactatccagatagcgtgaaaggcagattcactatttcccgcgacaatgcaaagaacaatctgtacctgcagatgagttcactgaggagcgaggataccgccctgtactattgcgctagatttgactatggaagctccctggattgttggggacaggggaccacactgaccgtgtctagt

SEQ ID NO: 255 - DNA, 321 bp, synthetic construct
  misc_feature 1..321: note = Synthetic Construct
  source 1..321: mol_type = other DNA
gacatcgtcctgactcagagccctgccaccctgtccgtgacaccaggcgattcagtcagcctgtcctgtagagcttctcagagtatctcaaactacctgcactggtatcagcagaagagtcatgaatcacccagactgctgatcaagtacgccagccagtccatctctgggattcctagccgcttcagtggctcaggaagcgggacagactttactctgagcatcaattccgtggagacagaagatttcggcatgtatttttgtcagcagtccaagtcttggcccaggacatttggcggagggactgagctggagatcaag

SEQ ID NO: 256 - DNA, 360 bp, synthetic construct
  misc_feature 1..360: note = Synthetic Construct
  source 1..360: mol_type = other DNA
gaggtgcaactggtgcagtctggagcagaggtgaaaaagcccggggagtctctgaagatctcctgtaagggttctggatacagctttaccagctactggatcggctgggtgcgccagatgcccgggaaaggcctggagtggatggggatcatctatcctggtgactctgataccagatacagcccgtccttccaaggccaggtcaccatctcagccgacaagtccatcagcaccgcctacctgcagtggagcagcctgaaggcctcggacaccgccatgtattactgtgcgagacgcgggtatcgcagcagctggtactttgactactggggccagggaaccctggtcaccgtctcctca

SEQ ID NO: 257 - DNA, 321 bp, synthetic construct
  misc_feature 1..321: note = Synthetic Construct
  source 1..321: mol_type = other DNA
gccatccagatgacccagtctccatcctccctgtctgcatctgtaggagacagagtcaccatcacttgccgggcaagtcagggcattagaaatgatttaggctggtatcagcagaaaccagggaaagcccctaagctcctgatctatgctgcatccagtttacaaagtggggtcccatcaaggttcagcggcagtggatcaggcacagatttcactttcaccatcagcagcctgcagcctgaagattttgcaacttattactgtctacaagattacaattacccgctcactttcggcggagggaccaaggtggagatcaaa

SEQ ID NO: 258 - DNA, 354 bp, synthetic construct
  misc_feature 1..354: note = Synthetic Construct
  source 1..354: mol_type = other DNA
gaggtgcagctggtggagtctgggggaggtgtggtacggccgggggggtccctgagactctcctgtgcagcctctggattcacctttgatgattatggcatgagctgggtccgccaagctccagggaaggggctggagtgggtctctggtattaattggaatggtggtagcacaggttatgcagactctgtgaagggccgattcaccatctccagagacaacgccaagaactccctgtatctgcaaatgaacagtctgagagccgaggacacggccttgtatcactgtgcgagagaagggggggagctattaatggactattggggccagggaaccctggtcaccgtctcctca

SEQ ID NO: 259 - DNA, 321 bp, synthetic construct
  misc_feature 1..321: note = Synthetic Construct
  source 1..321: mol_type = other DNA
gaaattgtgttgacacagtctccagccaccctgtctttgtctccaggggaaagagccaccctctcctgcagggccagtcagagtgttagcacctacttagcctggtaccaacagaaacctggccaggctcccaggctcctcatctatgatgcatccaacagggccactggcatcccacccaggttcagtggcagtgggtctgggacagacttcactctcaccatcagcagcctagagcctgaagattttgcagtttattactgtcagcagcgtagcaactggcctcctactttcggcggagggaccacggtggagatcaaa

SEQ ID NO: 260 - DNA, 375 bp, synthetic construct
  misc_feature 1..375: note = Synthetic Construct
  source 1..375: mol_type = other DNA
gaagttcaattgttagagtctggtggcggtcttgttcagcctggtggttctttacgtctttcttgcgctgcttccggattcactttctctcattactctatggtttgggttcgccaagctcctggtaaaggtttggagtgggtttcttatatctatccttctggtggcacttcgtatgctgactccgttaaaggtcgcttcactatctctagagacaactctaagaatactctctacttgcagatgaacagcttaagggctgaggacacggccgtgtattactgtgcgagacattggcgggggtatagcagcagctggtaccacccggcgtactttgactactggggccagggcaccctggtcaccgtctcaagc

SEQ ID NO: 261 - DNA, 321 bp, synthetic construct
  misc_feature 1..321: note = Synthetic Construct
  source 1..321: mol_type = other DNA
gacatccagatgacccagtctccagccaccctgtctttgtctccaggggaaagagccaccctctcctgcagggccagtcagagtgttagcagctacttagcctggtaccaacagaaacctggccaggctcccaggctcctcatctatgatgcatccaacagggccactggcatcccagccaggttcagtggcagtgggtctgggacagacttcactctcaccatcagcagcctagagcctgaagattttgcagtttattactgtcagcagcgtagcaactggcctctcactttcggcggagggaccaaggtggagatcaaa

SEQ ID NO: 262 - DNA, 378 bp, synthetic construct
  misc_feature 1..378: note = Synthetic Construct
  source 1..378: mol_type = other DNA
gaagttcaattgttagagtctggtggcggtcttgttcagcctggtggttctttacgtctttcttgcgctgcttccggattcactttctcttggtaccctatgatgtgggttcgccaagctcctggtaaaggtttggagtgggtttcttctatctatccttctggtggcactactacttatgctgactccgttaaaggtcgcttcactatctctagagacaactctaagaatactctctacttgcagatgaacagcttaagggctgaggacacggccgtgtattactgtgcgaggtcgtattactatgatagtagtggttattactcacatgatgcttttgatatctggggccaagggacaatggtcaccgtctcaagc

SEQ ID NO: 263 - DNA, 324 bp, synthetic construct
  misc_feature 1..324: note = Synthetic Construct
  source 1..324: mol_type = other DNA
gacatccagatgacccagtctccatcctccctgtctgcatctgtgggagacagagtcgccatcacttgccgcgcaagtcagagcatcgacacctatttaaattggtatcagcagaaaccagggaaagcccctaaactcctgatctatgctgcatccaagttggaagacggggtcccatcaagattcagtggcagtggaactgggacagatttcactctcaccatcagaagtctgcaacctgaagattttgcaagttatttctgtcaacagagctactctagtccagggatcactttcggccctgggaccaaggtggagatcaaa

SEQ ID NO: 264 - DNA, 366 bp, synthetic construct
  misc_feature 1..366: note = Synthetic Construct
  source 1..366: mol_type = other DNA
gaagttcaattgttagagtctggtggcggtcttgttcagcctggtggttctttacgtctttcttgcgctgcttccggattcactttctctgattacgagatgcattgggttcgccaagctcctggtaaaggtttggagtgggtttcttctatctggccttctggtggccttactaagtatgctgaccccgttaaaggtcgcttcactatctctagagacaactctaagaatactctctacttgcagatgaacagcttaagggctgaggacacggccgtgtattactgtgcgagagattcctattactatgatagtagtggtgctcttggctactggggccagggaaccctggtcaccgtctcaagc

SEQ ID NO: 265 - DNA, 321 bp, synthetic construct
  misc_feature 1..321: note = Synthetic Construct
  source 1..321: mol_type = other DNA
gacatccagatgacccagtctccttccaccctgtctgcatctgtaggagacagagtcaccatcacttgccgggccagtcagagtgttagtaactggttggcctggtatcagcagaaaccagggaaagcccctaagctcctgatctataaggcgtctagtttagaaagtggggtcccatcgaggttcagcggcagtggatctgggacagaattcactctcaccatcagcagcctgcagcctgatgattttgcaacttattactgcctacagtatgtgagttatcccctcacttttggcggagggaccaaggtggacatcaaa

SEQ ID NO: 266 - DNA, 372 bp, synthetic construct
  misc_feature 1..372: note = Synthetic Construct
  source 1..372: mol_type = other DNA
gaagttcaattgttagagtctggtggcggtcttgttcagcctggtggttctttacgtctttcttgcgctgcttccggattcactttctcttattacgatatgtattgggttcgccaagctcctggtaaaggtttggagtgggtttctcgtatctattcttctggtggccatacttggtatgctgactccgttaaaggtcgcttcactatctctagagacaactctaagaatactctctacttgcagatgaacagcttaagggctgaggacacggctgtgtattactgtgcgaggcccgggtatagcagtggctggtacgatggcacctactttgactactggggccagggaaccctggtcaccgtctcaagc

SEQ ID NO: 267 - DNA, 321 bp, synthetic construct
  misc_feature 1..321: note = Synthetic Construct
  source 1..321: mol_type = other DNA
gacatccagatgacccagtctccttccaccctgtctgcatctgttggcgacagagtcaccattacttgtcgggccagtcagagtattgatacttggctggcctggtatcggcagaaaccagggaaagcccctaatgtcgtaattcattccgcgtctactttacaaagtggcgtccccgcaaggttcagcggcagtggatttgggacagaatggactctcactatcaccaacctgcagcctgatgattttgccacctattattgccaacaatataagacttatccgttcacttttggccaggggacgaagctggagatcaag

SEQ ID NO: 268 - DNA, 357 bp, synthetic construct
  misc_feature 1..357: note = Synthetic Construct
  source 1..357: mol_type = other DNA
gaagttcaattgttagagtctggtggcggtcttgttcagcctggtggttctttacgtctttcttgcgctgcttccggattcactttctctcattaccagatggagtgggttcgccaagctcctggtaaaggtttggagtgggtttcttctatctctccttctggtggctttacttcttatgctgactccgttaaaggtcgcttcactatctctagagacaactctaagaatactctctacttgcagatgaacagcttaagggctgaggacacagccgtgtattactgtacgagagagccggggaggttgtgggcttttgatatctggggccaagggacaatggtcaccgtctcaagc

SEQ ID NO: 269 - DNA, 321 bp, synthetic construct
  misc_feature 1..321: note = Synthetic Construct
  source 1..321: mol_type = other DNA
gacatccagatgacccagtctccatctttcgtgtctgcatctgtcggagacagagtcaccatcacttgccgggcgagtcaggatattcgtaattggctagcctggtatcaacaggagtccgggaaagcccctcggctcctgatctctgctgcatccagtaggcacagtggcgtctcatctagattcagcggcagtggatctgggacagacttcaccctcaccatcaccagtctgcagcctgaagattcagcaacttatttttgtcaacaggctgacagttcccctcggacgttcggccaagggaccaaggtggaaatcaaa

SEQ ID NO: 270 - DNA, 345 bp, synthetic construct
  misc_feature 1..345: note = Synthetic Construct
  source 1..345: mol_type = other DNA
caggtgcaactggtgcagtctggggctgaggtgaagaagcctggggcctcagtgaaggtctcctgcaaggcttctggatacaccttcaccggctactatatgcactgggtgcgacaggcccctggacaagggcttgagtggatgggatggatcaaccctaacagtggtggcacaaactatgcacagaagtttcagggcagggtcaccatgaccagggacacgtccatcaacacagcctacatggaactgagcaggctgagatctgacgacacggccgtgtattactgtgcggtctttggttcggggagttcttggggccagggaaccctggtcaccgtctcctca

SEQ ID NO: 271 - DNA, 321 bp, synthetic construct
  misc_feature 1..321: note = Synthetic Construct
  source 1..321: mol_type = other DNA
gacatccagatgacccagtctccatcctcactgtctgcatctgtgggagacagagtcaccatcacttgtcgggcgagtcagggtattagcaattctttagcctggtttcagcagaaaccagggaaagcccctaagtccctgatctatgctgcatccagtttgcaaagtggggtcccatcaaagttcagcggcagtggatctgggacagatttcactctcaccatcagcagcctgcagcctgaagattttgcaacttattactgccaacaatataagagttacccgtacacatttggccaggggaccaagctggagatcaaa

SEQ ID NO: 272 - DNA, 345 bp, synthetic construct
  misc_feature 1..345: note = Synthetic Construct
  source 1..345: mol_type = other DNA
caggtgcagctggtgcagtctggggctgaggtgaagaagcctggggcctcagtgaaggtctcctgcaaggcttctggaaacaccttcaccggctactatatacactgggttcgacaggcccctggacaagggcttgagtggatgggatggattaaacctagtactggtgacacaaactatgcacagaattttctggacagggtcaccatgaccagggacacgtccatcagcacagcctacatggaactcagcaggctgagatctgacgacacggccgtgtattactgtgcggtctttggttcggggagttcttggggccagggaaccctggtcaccgtctcctca

SEQ ID NO: 273 - DNA, 321 bp, synthetic construct
  misc_feature 1..321: note = Synthetic Construct
  source 1..321: mol_type = other DNA
gacatccacatgacccagtctccatcctcactgtctgcatttgtaggagacagagtcaccatcacttgtcgggcgagtcagggcattagcaattatttagcctggtttcagcagaaaccagggaaagcccctaagtccctgatctatgctgcatccagtttgcaaagtggggtcccatcaaagttcagcggcagtggatctgggacagatttcactctcaccatcaacaacctgcagcctgaagattttgcaacttattactgccaacagtataagacttacccgtacacatttggccaggggaccaagctggagatcaaa

SEQ ID NO: 274 - DNA, 372 bp, synthetic construct
  misc_feature 1..372: note = Synthetic Construct
  source 1..372: mol_type = other DNA
caggtgcagctggtggagtctgggggaggcgtggtccagcctgggaggtccctgagactctcctgtgcagcgtctggattcaccttcagtagctatggcatgcactgggtccgccaggctccaggcaaggggctggagtgggtggcagttatatggtatgatggaagtaataaatactatgcagactccgtgaagggccgattcaccatctccagagacaattccaagaacacgctgtatctgcaaatgaacagtctgagagccgaggacgcggctgtgtattactgtgcgagagaaggtggctggtacggcggggactactactacggtatggacgtctggggccaagggaccacggtcaccgtctcctca

SEQ ID NO: 275 - DNA, 321 bp, synthetic construct
  misc_feature 1..321: note = Synthetic Construct
  source 1..321: mol_type = other DNA
gccatccagttgacccagtctccatcctccctgtctgcatctgtaggagacagagtcaccatcacttgccgggcaagtcagggcattagcagtgctttagcctggtatcagcagaaaccagggaaagctcctaagctcctgatctatgatgcctccagtttggaaagtggggtcccatcaaggttcagcggcagtggatctgggacagatttcactctcaccatcagcagcctgcagcctgaagattttgcaacttattactgtcatcagtttaataattacccattcactttcggccctgggaccaaagtggatatcaaa

SEQ ID NO: 276 - DNA, 366 bp, synthetic construct
  misc_feature 1..366: note = Synthetic Construct
  source 1..366: mol_type = other DNA
gaagtgcagctgctggaatctggcggcggactggtgcagcctggcggatctctgagactgtcctgtgtggcctccggcttcaccttctccagctacgccatgtcctgggtgcgacaggctcctggcaagggcctggaatgggtgtccggcatctctggcaggggcggctctcctaactacgccgactctgtgaagggccggttcaccatctcccgggacaactccaagaacaccctgtacctccagatgaactccctgcgggccgaggacaccgccgtgtactactgtgctaaggacggcgacggctccggccctccctactactttgattactggggccagggcaccctcgtgaccgtgtcatct

SEQ ID NO: 277 - DNA, 321 bp, synthetic construct
  misc_feature 1..321: note = Synthetic Construct
  source 1..321: mol_type = other DNA
gacatccagatgacccagtccccctccagcctgtctgcctctgtgggcgacagagtgaccatcacctgtcgggcctcccagggcatctcttcttggctggcctggtatcagcagaagcccgagaaggcccccaagtccctgatctacgccgccagctctctccagtctggcgtgccctccagattctccggctctggctctggcaccgactttaccctgaccatcagctccctccagcccgaggacttcgccacctactactgccagcagtacaactcctacccctacaccttcggccagggcaccaagctggaaatcaag

SEQ ID NO: 278 - DNA, 393 bp, synthetic construct
  misc_feature 1..393: note = Synthetic Construct
  source 1..393: mol_type = other DNA
caggtgcagctgatggagtctgggggaggcgtggtccagcctgggaggtccctgagactctcctgtgcagcgtctggattcaccttcagtggctatggcatgcactgggtccgccaggctccagggaaggggctggagtgggtggcagttatatggtctgatggaagtaatagatactatacagactccgtgaagggccgattcaccatctccagagacaattccaagaacacgctgtctctgcaaatgaacagcctgagagccgaggacacggctgtgtattactgtgcgagagatagggggattactatggttcggggacttattataaaatactactactactacggtttggacgtctggggccaagggacctcggtcaccgtctcctca

SEQ ID NO: 279 - DNA, 318 bp, synthetic construct
  misc_feature 1..318: note = Synthetic Construct
  source 1..318: mol_type = other DNA
gaaattgtgttgacacagtctccagccaccctgtctttgtctccaggggaaagagccaccctctcctgcagggccagtcagagtgttagcagctacttagcctggtaccaacagaaacctggccaggctcccaggctcctcatctatgatgcatccaacagggccactggcatcccagccaggttcagtggcagtgggtctgggacagacttcactctcaccatcagcagcctagagcctgaagattttgcagtttattactgtcagcagcgtagcaactggtggacgttcggccaagggaccaaggtggaaatcaaa

SEQ ID NO: 280 - DNA, 360 bp, synthetic construct
  misc_feature 1..360: note = Synthetic Construct
  source 1..360: mol_type = other DNA
caggtgcagctggtggagtctgggggaggcgtggtccagcctgggaggtccctgagactctcctgtgcagcgtctggattcaccttcagtagctttggcatgcactgggtccgccaggctccaggcaaggggctggagtgggtggcagttatatactatgatggaagtaataaatactatgcagactccgtgaagggccgattcaccatctccagagacaattccaagaacacgctgtatctgcaaatgaacagcctgagagccgaggacacggctgtgtattactgtgcgagagatgacaactggaacgacggggactttgactactggggccagggaaccctggtcaccgtctcctca

SEQ ID NO: 281 - DNA, 321 bp, synthetic construct
  misc_feature 1..321: note = Synthetic Construct
  source 1..321: mol_type = other DNA
gacatccagttgacccagtctccatccttcctgtctgcatctgtaggagacagagtcaccatcacttgccgggccagtcagggcattagtagttatttagcctggtatcagcaaaaaccagggaaagcccctaagctcctgatctatgctgcatccactttgcaaagtggggtcccatcaaggttcagcggcagtggatctgggacagaattcactctcacaatcagcagcctgcagcctgaagattttgcaacttattactgtcaacagcttaatagttaccctcggacgttcggccaagggaccaaggtggaaatcaaa

SEQ ID NO: 282 - DNA, 378 bp, synthetic construct
  misc_feature 1..378: note = Synthetic Construct
  source 1..378: mol_type = other DNA
gaggtgcagctgttggagtctgggggaggcttggtacagcctggggagtccctgagactctcctgtgcagcctctggattcacctttaacagatttgtcatgagttgggtccgccaggctccagggaaggggctggagtgggtctcaactattagtggtagtggtggtagcacatactacgcagactccgtgaagggccggttcaccatctccagagacaattccaagaacacgctgtatctgcaaatgaacagcctgagagccgaggacacggccgtgtattactgtgcgaaagattttacgtattactatggttcggggaattattataactggttcgaccccaggggccagggaaccctggtcaccgtctcctca

SEQ ID NO: 283 - DNA, 321 bp, synthetic construct
  misc_feature 1..321: note = Synthetic Construct
  source 1..321: mol_type = other DNA
gacatccagatgacccagtctccttccaccctgtctacatctgtaggagacagagtcaccatcacttgccgggccagtcagagtattagtagctggttggcctggtatcagcagaaaccagggaaagcccctaagctcctgatctataaggcgtctagtttagaaagtggggtcccatcaaggttcagcggcagtggatctgggacagaattcactctcaccatcagcagcctgcagcctgatgattttgcaacttattactgccaacagtataatagttattctcggacgttcggccaagggaccaaggtggaaatcaaa

SEQ ID NO: 284 - DNA, 363 bp, synthetic construct
  misc_feature 1..363: note = Synthetic Construct
  source 1..363: mol_type = other DNA
caggtgcagctacagcagtggggcgcaggactgttgaagccttcggagaccctgtccctcacctgcgctgtctatggtgggtcctttagtggttactactggagctggatccgccagcccccagggaaggggctggagtggattggggaaatcaatcatagtggaggcaccaactacaacccgtccctcaagagtcgagtcaccatatcagtagacacgtccaagaaccacttctccctgaagctgagctctgtgaccgccgcggacacggctgtgtattactgtgcgagaactagtgactacgattactactactacggtatggacgtctggggccaagggaccacggtcaccgtctcctca

SEQ ID NO: 285 - DNA, 348 bp, synthetic construct
  misc_feature 1..348: note = Synthetic Construct
  source 1..348: mol_type = other DNA
cagcctgtgctgactcagccaacttccctctcagcatctcctggagcatcagccagactcacctgcaccttgcgcagtggcatcaatcttggtcgctacaggatattctggtaccagcagaagccagagagccctccccggtatctcctgagctactactcagactcaagtaagcatcagggctctggagtccccagccgcttctctggatccaaagatgcttcgagcaatgcagggattttagtcatctctgggctccagtctgaggatgaggctgactattactgtatgatttggcacaggagtgctttgtttattttcggcagtggaaccaaggtcactgtccta

SEQ ID NO: 286 - DNA, 345 bp, synthetic construct
  misc_feature 1..345: note = Synthetic Construct
  source 1..345: mol_type = other DNA
caggttcagctacagcagtctggacctgagctggtgaagcctggggcttcagtgaagttgtcctgcaaggcttctggttacaccttcacaagctacgagataaactggttgaagcagaggcctggacagggacttgagtggattggattgatttatcctagagatggagatactaagtacaatgagaagttcaagggcaaggccacattgactgcagacacatcctccagcacagcgtacatggagctccacagcctgacatctgaggactctgcggtctatttctgtgcaagacacaccccaggggctttctggggccaagggactctggtcactgtctctgca

SEQ ID NO: 287 - DNA, 336 bp, synthetic construct
  misc_feature 1..336: note = Synthetic Construct
  source 1..336: mol_type = other DNA
gatgttgtgatgacccaaactcccctctccctgccggtcagtcttggagatcaagcctccatctcttgcagatctagtcagagccttgttcacagtaatggagacacctatttacattggtacctacagaagccaggccagtctccaaagctcctgatctacaaagtttccaaccgattttctggggtcccagacaggttcagtggcagtggatcagggacagatttcacactcaagatcagcagagtggaggctgaggatctggaaatttatttctgctctcaaagcacacatgttccgtacacgttcggaggggggaccaaactggaaataaaa

SEQ ID NO: 288 - DNA, 372 bp, synthetic construct
  misc_feature 1..372: note = Synthetic Construct
  source 1..372: mol_type = other DNA
gacgtgaagctggtggagtctggggaaggcttagtgaagcccggagggtccctgaaactctcttgtgcagcctctggattcactttcagtaggtatgccatgtcttgggttcgccagactccagaaaagaggctggaatgggtcgcatatattagtagtggaggtgattacatccactatggagaaactgtgaagggccgattcaccatctccagagacaatgccaggaacaccctgtacctgcaaatgagcagtctgaagtctgaggacacagccatgtattactgtacaagagttctcttttattattacggcagtagctacgtcttttttgactactggggccaaggcaccactctcacagtctcctca

SEQ ID NO: 289 - DNA, 321 bp, synthetic construct
  misc_feature 1..321: note = Synthetic Construct
  source 1..321: mol_type = other DNA
gatatccagatgacacagactacatcctccctgtcagtctctctgggagacagagtcaccatcagttgcagggcaagtcaggacatcagcaattttctaaactggtatcagcagaaaccagatggaactgttaatctcctgatctactacacatcaaaattacactcaggagtcccatcaaggttcagtggcggtgggtctggaagagattattctctcaccattaataacctggagcaagaagatattgcctcttacttttgccaacagggtcatacgcttccgtatacgttcggaggggggaccaagctggaaataaaa

SEQ ID NO: 290 - protein, 95 aa, synthetic construct
  REGION 1..95: note = Synthetic Construct
SIVVEWTNNTLPLEPCPKEQIIGLSRRIADENGKPRPAFSNALEPDFKALSIAVTGSGSCRHLQFIPVAPPSPGSSAAPATEVPDRDPEKSSEDD

SEQ ID NO: 291 - protein, 96 aa, synthetic construct
  REGION 1..96: note = Synthetic Construct
SIVVEWTNNTLPLEPCPKEQIAGLSRRIAEDDGKPRPAFSNALEPDFKATSITVTGSGSCRHLQFIPVVPPRRVPSEAPPTEVPDRDPEKSSEDDV

SEQ ID NO: 292 - protein, 183 aa, synthetic construct
  REGION 1..183: note = Synthetic Construct
ANAESGTYFDGTGFAKAVGGFKVGLDLLVEFEFRTWTGVLLGVSSQKMDGMGIEMIDEKLMFHVDNGAGRFTAIYDAGIPGHMCNGQWHKVTAKKIKNRLELVVDGNQVDAQSPNSASTSADTNDPVFVGGFPGQQFGLTTNIRFRGCIRSLKLTKGTGKPLEVNFAKALELRGVQPVSCPTT

SEQ ID NO: 293 - protein, 187 aa, synthetic construct
  REGION 1..187: note = Synthetic Construct
ANAQRGTYFDGTGFAKAVGGFKVGLDLLVEFEFRTTTTTGVLLGISSQKMDGMGIEMIDEKLMFHVDNGAGRFTAVYDAGVPGHLCDGQWHKVTANKIKHRIELTVDGNQVEAQSPNPASTSADTNDPVFVGGFPDDLKQFGLTTSIPFRGCIRSLKLTKGTGKPLEVNFAKALELRGVQPVSCPAN

SEQ ID NO: 294 - protein, 10 aa, synthetic construct
  REGION 1..10: note = Synthetic Construct
GGGGSGGGGS

SEQ ID NO: 295 - protein, 20 aa, synthetic construct
  REGION 1..20: note = Synthetic Construct
GFAKAVGGFKVGLDLLVEFE

SEQ ID NO: 296 - protein, 14 aa, synthetic construct
  REGION 1..14: note = Synthetic Construct
EPKSDKTHTSPPSP

SEQ ID NO: 297 - protein, 7 aa, synthetic construct
  REGION 1..7: note = Synthetic Construct
GQPKAAP

SEQ ID NO: 298 - protein, 5 aa, synthetic construct
  REGION 1..5: note = Synthetic Construct
TKGPS

SEQ ID NO: 299 - protein, 10 aa, synthetic construct
  REGION 1..10: note = Synthetic Construct
GGSGSSGSGG

SEQ ID NO: 300 - protein, 390 aa, synthetic construct
  REGION 1..390: note = Synthetic Construct
VQPQPVPTPAFPFPAPTMVHGPCVAESEPALLTGSKQFGLSRNSHIAIAFDDTKVKNRLTIELEVRTEAESGLLFYMARINHADFATVQLRNGFPYFSYDLGSGDTSTMIPTKINDGQWHKIKIVRVKQEGILYVDDASSQTISPKKADILDVVGILYVGGLPINYTTRRIGPVTYSLDGCVRNLHMEQAPVDLDQPTSSFHVGTCFANAESGTYFDGTGFAKAVGGFKVGLDLLVEFEFRTWTGVLLGVSSQKMDGMGIEMIDEKLMFHVDNGAGRFTAIYDAGIPGHMCNGQWHKVTAKKIKNRLELVVDGNQVDAQSPNSASTSADTNDPVFVGGFPGQQFGLTTNIRFRGCIRSLKLTKGTGKPLEVNFAKALELRGVQPVSCPTT

SEQ ID NO: 301 - protein, 391 aa, synthetic construct
  REGION 1..391: note = Synthetic Construct
QPEPVPTPAFPTPTPVLTHGPCAAESEPALLIGSKQFGLSRNSHIAIAFDDTKVKNRLTIELEVRTEAESGLLFYMARINHADFATVQLRNGLPYFSYDLGSGDTHTMIPTKINDGQWHKIKIMRSKQEGILYVDGNRTISPKKADILDVVGMLYVGGLPINYTTRRIGPVTYSIDGCVRNLHMAEAPADLEQPTSSFHVGTCFANAQRGTYFDGTGFAKAVGGFKVGLDLLVEFEFRTTTTTGVLLGISSQKMDGMGIEMIDEKLMFHVDNGAGRFTAVYDAGVPGHLCDGQWHKVTANKIKHRIELTVDGNQVEAQSPNPASTSADTNDPVFVGGFPDDLKQFGLTTSIPFRGCIRSLKLTKGTGKPLEVNFAKALELRGVQPVSCPAN

SEQ ID NO: 302 - protein, 11 aa, synthetic construct
  REGION 1..11: note = Synthetic Construct
DRDPEKSSEDD

SEQ ID NO: 303 - protein, 180 aa, synthetic construct
  REGION 1..180: note = Synthetic Construct
GDRAPARFKAKFVGDPALVLNDIHKKIALVKKLAFAFGDRNCSTITLQNITRGSIVVEWTNNTLPLEPCPKEQIAGLSRRIAEDDGKPRPAFSNALEPDFKATSITVTGSGSCRHLQFIPVVPPRRVPSEAPPTEVPDRDPEKSSEDDVYLHTVIPAVVVAAILLIAGIIAMICYRKKRK

SEQ ID NO: 304 - protein, 180 aa, synthetic construct
  REGION 1..180: note = Synthetic Construct
GDKAPARFKARLAGDPAPVVNDIHKKIALVKKLAFAFGDRNCSSITLQNITRGSIVVEWTNNTLPLEPCPKEQIIGLSRRIADENGKPRPAFSNALEPDFKALSIAVTGSGSCRHLQFIPVAPPSPGSSAAPATEVPDRDPEKSSEDDVYLHTVIPAVVVAAILLIAGIIAMICYRKKRK

SEQ ID NO: 305 - protein, 392 aa, synthetic construct
  REGION 1..392: note = Synthetic Construct
IQPEPVPTPAFPTPTPVLTHGPCAAESEPALLIGSKQFGLSRNSHIAIAFDDTKVKNRLTIELEVRTEAESGLLFYMARINHADFATVQLRNGLPYFSYDLGSGDTHTMIPTKINDGQWHKIKIMRSKQEGILYVDGNRTISPKKADILDVVGMLYVGGLPINYTTRRIGPVTYSIDGCVRNLHMAEAPADLEQPTSSFHVGTCFANAQRGTYFDGTGFAKAVGGFKVGLDLLVEFEFRTTTTTGVLLGISSQKMDGMGIEMIDEKLMFHVDNGAGRFTAVYDAGVPGHLCDGQWHKVTANKIKHRIELTVDGNQVEAQSPNPASTSADTNDPVFVGGFPDDLKQFGLTTSIPFRGCIRSLKLTKGTGKPLEVNFAKALELRGVQPVSCPAN

SEQ ID NO: 306 - DNA, 339 bp, synthetic construct
  misc_feature 1..339: note = Synthetic Construct
  source 1..339: mol_type = other DNA
caagtacaactggttcaatcaggcgcagaagtcgtaaaacctggttccagcgtaaaagtcagttgtgaggctagtggattcaccttcaccgatagcgttattacatgggttcgtcagcgcccaggtcaagggctcgagtggattggggaaatttacccaggaagtggaaatttctactacaatgaaaaatttcaaggccgggtgaccatcactgctgataaaagcacttcaacagcctatatggaattgtccagcttgcgctccgaagacactgccgtttatttctgcgccatgcgtaggtcttcctggggacagggtacacttgtaactgtcagctct

SEQ ID NO: 307 - DNA, 75 bp, synthetic construct
  misc_feature 1..75: note = Synthetic Construct
  source 1..75: mol_type = other DNA
caagtacaactggttcaatcaggcgcagaagtcgtaaaacctggttccagcgtaaaagtcagttgtgaggctagt

SEQ ID NO: 308 - DNA, 24 bp, synthetic construct
  misc_feature 1..24: note = Synthetic Construct
  source 1..24: mol_type = other DNA
ggattcaccttcaccgatagcgtt

SEQ ID NO: 309 - DNA, 51 bp, synthetic construct
  misc_feature 1..51: note = Synthetic Construct
  source 1..51: mol_type = other DNA
attacatgggttcgtcagcgcccaggtcaagggctcgagtggattggggaa

SEQ ID NO: 310 - DNA, 24 bp, synthetic construct
  misc_feature 1..24: note = Synthetic Construct
  source 1..24: mol_type = other DNA
atttacccaggaagtggaaatttc

SEQ ID NO: 311 - DNA, 114 bp, synthetic construct
  misc_feature 1..114: note = Synthetic Construct
  source 1..114: mol_type = other DNA
tactacaatgaaaaatttcaaggccgggtgaccatcactgctgataaaagcacttcaacagcctatatggaattgtccagcttgcgctccgaagacactgccgtttatttctgc

SEQ ID NO: 312 - DNA, 18 bp, synthetic construct
  misc_feature 1..18: note = Synthetic Construct
  source 1..18: mol_type = other DNA
gccatgcgtaggtcttcc

SEQ ID NO: 313 - DNA, 33 bp, synthetic construct
  misc_feature 1..33: note = Synthetic Construct
  source 1..33: mol_type = other DNA
tggggacagggtacacttgtaactgtcagctct

SEQ ID NO: 314 - protein, 113 aa, synthetic construct
  REGION 1..113: note = Synthetic Construct
QVQLVQSGAEVVKPGSSVKVSCEASGFTFTDSVITWVRQRPGQGLEWIGEIYPGSGNFYYNEKFQGRVTITADKSTSTAYMELSSLRSEDTAVYFCAMRRSSWGQGTLVTVSS

SEQ ID NO: 315 - protein, 25 aa, synthetic construct
  REGION 1..25: note = Synthetic Construct
QVQLVQSGAEVVKPGSSVKVSCEAS

SEQ ID NO: 316 - protein, 8 aa, synthetic construct
  REGION 1..8: note = Synthetic Construct
GFTFTDSV

SEQ ID NO: 317 - protein, 17 aa, synthetic construct
  REGION 1..17: note = Synthetic Construct
ITWVRQRPGQGLEWIGE

SEQ ID NO: 318 - protein, 8 aa, synthetic construct
  REGION 1..8: note = Synthetic Construct
IYPGSGNF

SEQ ID NO: 319 - protein, 38 aa, synthetic construct
  REGION 1..38: note = Synthetic Construct
YYNEKFQGRVTITADKSTSTAYMELSSLRSEDTAVYFC

SEQ ID NO: 320 - protein, 6 aa, synthetic construct
  REGION 1..6: note = Synthetic Construct
AMRRSS

SEQ ID NO: 321 - protein, 11 aa, synthetic construct
  REGION 1..11: note = Synthetic Construct
WGQGTLVTVSS

SEQ ID NO: 322 - DNA, 336 bp, synthetic construct
  misc_feature 1..336: note = Synthetic Construct
  source 1..336: mol_type = other DNA
gacgtcgtaatgactcaaacacccctctctctttctgttacccccggacagcctgcttcaatcagttgtaaatcatcccaaaccatagttcattctaatagtaaaacttacctcgaatggtatctccaaaaacctggtcagtcaccacagctccttatttacaaggttagttccagattctctggcgtccctgaccgcttctctggctccggttcaggcaccgactttactctgaaaatctcacgggttgaagctgaagatgttggagtgtactactgcttccagggttctcacgtcccattgacctttggacagggaactaagctcgaaataaaa

SEQ ID NO: 323 - DNA, 78 bp, synthetic construct
  misc_feature 1..78: note = Synthetic Construct
  source 1..78: mol_type = other DNA
gacgtcgtaatgactcaaacacccctctctctttctgttacccccggacagcctgcttcaatcagttgtaaatcatcc

SEQ ID NO: 324 - DNA, 33 bp, synthetic construct
  misc_feature 1..33: note = Synthetic Construct
  source 1..33: mol_type = other DNA
caaaccatagttcattctaatagtaaaacttac

SEQ ID NO: 325 - DNA, 51 bp, synthetic construct
  misc_feature 1..51: note = Synthetic Construct
  source 1..51: mol_type = other DNA
ctcgaatggtatctccaaaaacctggtcagtcaccacagctccttatttac

SEQ ID NO: 326 - skipped

SEQ ID NO: 327 - DNA, 108 bp, synthetic construct
  misc_feature 1..108: note = Synthetic Construct
  source 1..108: mol_type = other DNA
tccagattctctggcgtccctgaccgcttctctggctccggttcaggcaccgactttactctgaaaatctcacgggttgaagctgaagatgttggagtgtactactgc

SEQ ID NO: 328 - DNA, 27 bp, synthetic construct
  misc_feature 1..27: note = Synthetic Construct
  source 1..27: mol_type = other DNA
ttccagggttctcacgtcccattgacc

SEQ ID NO: 329 - DNA, 30 bp, synthetic construct
  misc_feature 1..30: note = Synthetic Construct
  source 1..30: mol_type = other DNA
tttggacagggaactaagctcgaaataaaa

SEQ ID NO: 330 - protein, 112 aa, synthetic construct
  REGION 1..112: note = Synthetic Construct
DVVMTQTPLSLSVTPGQPASISCKSSQTIVHSNSKTYLEWYLQKPGQSPQLLIYKVSSRFSGVPDRFSGSGSGTDFTLKISRVEAEDVGVYYCFQGSHVPLTFGQGTKLEIK

SEQ ID NO: 331 - protein, 26 aa, synthetic construct
  REGION 1..26: note = Synthetic Construct
DVVMTQTPLSLSVTPGQPASISCKSS

SEQ ID NO: 332 - protein, 11 aa, synthetic construct
  REGION 1..11: note = Synthetic Construct
QTIVHSNSKTY

SEQ ID NO: 333 - protein, 17 aa, synthetic construct
  REGION 1..17: note = Synthetic Construct
LEWYLQKPGQSPQLLIY

SEQ ID NO: 334 - skipped

SEQ ID NO: 335 - protein, 36 aa, synthetic construct
  REGION 1..36: note = Synthetic Construct
SRFSGVPDRFSGSGSGTDFTLKISRVEAEDVGVYYC

SEQ ID NO: 336 - protein, 9 aa, synthetic construct
  REGION 1..9: note = Synthetic Construct
FQGSHVPLT

SEQ ID NO: 337 - protein, 10 aa, synthetic construct
  REGION 1..10: note = Synthetic Construct
FGQGTKLEIK

SEQ ID NO: 338 - DNA, 339 bp, synthetic construct; identical to SEQ ID NO: 306
  misc_feature 1..339: note = Synthetic Construct
  source 1..339: mol_type = other DNA

SEQ ID NO: 339 - DNA, 75 bp, synthetic construct; identical to SEQ ID NO: 307
  misc_feature 1..75: note = Synthetic Construct
  source 1..75: mol_type = other DNA

SEQ ID NO: 340 - DNA, 24 bp, synthetic construct
  misc_feature 1..24: note = Synthetic Construct
  source 1..24: mol_type = other DNA
ggattcaccttcaccgatagcgtt

SEQ ID NO: 341 - DNA, 51 bp, synthetic construct; identical to SEQ ID NO: 309
  misc_feature 1..51: note = Synthetic Construct
  source 1..51: mol_type = other DNA

SEQ ID NO: 342 - DNA, 24 bp, synthetic construct
  misc_feature 1..24: note = Synthetic Construct
  source 1..24: mol_type = other DNA
atttacccaggaagtggaaatttc

SEQ ID NO: 343 - DNA, 114 bp, synthetic construct; identical to SEQ ID NO: 311
  misc_feature 1..114: note = Synthetic Construct
  source 1..114: mol_type = other DNA

SEQ ID NO: 344 - DNA, 18 bp, synthetic construct
  misc_feature 1..18: note = Synthetic Construct
  source 1..18: mol_type = other DNA
gccatgcgtaggtcttcc

SEQ ID NO: 345 - DNA, 33 bp, synthetic construct; identical to SEQ ID NO: 313
  misc_feature 1..33: note = Synthetic Construct
  source 1..33: mol_type = other DNA

SEQ ID NO: 346 - protein, 113 aa, synthetic construct; identical to SEQ ID NO: 314
  REGION 1..113: note = Synthetic Construct

SEQ ID NO: 347 - protein, 25 aa, synthetic construct
  REGION 1..25: note = Synthetic Construct
QVQLVQSGAEVVKPGSSVKVSCEAS

SEQ ID NO: 348 - protein, 8 aa, synthetic construct
  REGION 1..8: note = Synthetic Construct
GFTFTDSV

SEQ ID NO: 349 - protein, 17 aa, synthetic construct
  REGION 1..17: note = Synthetic Construct
ITWVRQRPGQGLEWIGE

SEQ ID NO: 350 - protein, 8 aa, synthetic construct
  REGION 1..8: note = Synthetic Construct
IYPGSGNF

SEQ ID NO: 351 - protein, 38 aa, synthetic construct; identical to SEQ ID NO: 319
  REGION 1..38: note = Synthetic Construct

SEQ ID NO: 352 - protein, 6 aa, synthetic construct
  REGION 1..6: note = Synthetic Construct
AMRRSS

SEQ ID NO: 353 - protein, 11 aa, synthetic construct
  REGION 1..11: note = Synthetic Construct
WGQGTLVTVSS

SEQ ID NO: 354 - DNA, 336 bp, synthetic construct
  misc_feature 1..336: note = Synthetic Construct
  source 1..336: mol_type = other DNA
gatgtggtgatgactcagacacccctgagtctcagcgtaacacctggtcaacccgcctctattagttgtcgaagctctcaaacaatcgtacatagtaatagtaaaacctatctcgaatggtatcttcagaaaccagggcagtctcctcaactccttatatacaaagtatccaacaggttttccggtgtacccgataggttttccggttccggctccggaactgactttaccctcaaaataagtcgagtggaggctgaggatgttggcgtttattattgctttcaggggtcacacgtacctcttaccttcggcgcaggcacaaaattggagattaaa

SEQ ID NO: 355 - DNA, 78 bp, synthetic construct
  misc_feature 1..78: note = Synthetic Construct
  source 1..78: mol_type = other DNA
gatgtggtgatgactcagacacccctgagtctcagcgtaacacctggtcaacccgcctctattagttgtcgaagctct

SEQ ID NO: 356 - DNA, 33 bp, synthetic construct
  misc_feature 1..33: note = Synthetic Construct
  source 1..33: mol_type = other DNA
caaacaatcgtacatagtaatagtaaaacctat

SEQ ID NO: 357 - DNA, 51 bp, synthetic construct
  misc_feature 1..51: note = Synthetic Construct
  source 1..51: mol_type = other DNA
ctcgaatggtatcttcagaaaccagggcagtctcctcaactccttatatac

SEQ ID NO: 358 - skipped

SEQ ID NO: 359 - DNA, 108 bp, synthetic construct
  misc_feature 1..108: note = Synthetic Construct
  source 1..108: mol_type = other DNA
aacaggttttccggtgtacccgataggttttccggttccggctccggaactgactttaccctcaaaataagtcgagtggaggctgaggatgttggcgtttattattgc

SEQ ID NO: 360 - DNA, 27 bp, synthetic construct
  misc_feature 1..27: note = Synthetic Construct
  source 1..27: mol_type = other DNA
tttcaggggtcacacgtacctcttacc

SEQ ID NO: 361 - DNA, 30 bp, synthetic construct
  misc_feature 1..30: note = Synthetic Construct
  source 1..30: mol_type = other DNA
ttcggcgcaggcacaaaattggagattaaa

SEQ ID NO: 362 - protein, 112 aa, synthetic construct
  REGION 1..112: note = Synthetic Construct
DVVMTQTPLSLSVTPGQPASISCRSSQTIVHSNSKTYLEWYLQKPGQSPQLLIYKVSNRFSGVPDRFSGSGSGTDFTLKISRVEAEDVGVYYCFQGSHVPLTFGAGTKLEIK

SEQ ID NO: 363 - protein, 26 aa, synthetic construct
  REGION 1..26: note = Synthetic Construct
DVVMTQTPLSLSVTPGQPASISCRSS

SEQ ID NO: 364 - protein, 11 aa, synthetic construct
  REGION 1..11: note = Synthetic Construct
QTIVHSNSKTY

SEQ ID NO: 365 - protein, 17 aa, synthetic construct
  REGION 1..17: note = Synthetic Construct
LEWYLQKPGQSPQLLIY

SEQ ID NO: 366 - skipped

SEQ ID NO: 367 - protein, 36 aa, synthetic construct
  REGION 1..36: note = Synthetic Construct
NRFSGVPDRFSGSGSGTDFTLKISRVEAEDVGVYYC

SEQ ID NO: 368 - protein, 9 aa, synthetic construct
  REGION 1..9: note = Synthetic Construct
FQGSHVPLT

SEQ ID NO: 369 - protein, 10 aa, synthetic construct
  REGION 1..10: note = Synthetic Construct
FGAGTKLEIK

SEQ ID NO: 370 - DNA, 354 bp, synthetic construct
  misc_feature 1..354: note = Synthetic Construct
  source 1..354: mol_type = other DNA
gaagttcaactggtcgagtctggaggaggcctcgtgaagccgggcggtagtttgcgcctctcttgtgccgcctcagggtttacgttctctagttatactatgagttgggtgcggcaggcaccgggaaaagggctggaatgggtggcctcaatctctagtagcggcagcaatacttattatcctgatagtgtgaaggggaggtttaccatctcacgggataacgctaagaacaacctgtatcttcaaatgaatagcctccgagcagaggatacagcactttactactgcgctcgctttgactatggcagcagtcttgatagttgggggcagggcaccttgcttacggtttcatcc

SEQ ID NO: 371 - DNA, 75 bp, synthetic construct
  misc_feature 1..75: note = Synthetic Construct
  source 1..75: mol_type = other DNA
gaagttcaactggtcgagtctggaggaggcctcgtgaagccgggcggtagtttgcgcctctcttgtgccgcctca

SEQ ID NO: 372 - DNA, 24 bp, synthetic construct
  misc_feature 1..24: note = Synthetic Construct
  source 1..24: mol_type = other DNA
gggtttacgttctctagttatact

SEQ ID NO: 373 - DNA, 51 bp, synthetic construct
  misc_feature 1..51: note = Synthetic Construct
  source 1..51: mol_type = other DNA
atgagttgggtgcggcaggcaccgggaaaagggctggaatgggtggcctca

SEQ ID NO: 374 - DNA, 24 bp, synthetic construct
  misc_feature 1..24: note = Synthetic Construct
  source 1..24: mol_type = other DNA
atctctagtagcggcagcaatact

SEQ ID NO: 375 - DNA, 114 bp, synthetic construct
  misc_feature 1..114: note = Synthetic Construct
  source 1..114: mol_type = other DNA
tattatcctgatagtgtgaaggggaggtttaccatctcacgggataacgctaagaacaacctgtatcttcaaatgaatagcctccgagcagaggatacagcactttactactgc

SEQ ID NO: 376 - DNA, 33 bp, synthetic construct
  misc_feature 1..33: note = Synthetic Construct
  source 1..33: mol_type = other DNA
gctcgctttgactatggcagcagtcttgatagt

SEQ ID NO: 377 - DNA, 33 bp, synthetic construct
  misc_feature 1..33: note = Synthetic Construct
  source 1..33: mol_type = other DNA
tgggggcagggcaccttgcttacggtttcatcc

SEQ ID NO: 378 - protein, 118 aa, synthetic construct
  REGION 1..118: note = Synthetic Construct
EVQLVESGGGLVKPGGSLRLSCAASGFTFSSYTMSWVRQAPGKGLEWVASISSSGSNTYYPDSVKGRFTISRDNAKNNLYLQMNSLRAEDTALYYCARFDYGSSLDSWGQGTLLTVSS

SEQ ID NO: 379 - protein, 25 aa, synthetic construct
  REGION 1..25: note = Synthetic Construct
EVQLVESGGGLVKPGGSLRLSCAAS

SEQ ID NO: 380 - protein, 8 aa, synthetic construct
  REGION 1..8: note = Synthetic Construct
GFTFSSYT

SEQ ID NO: 381 - protein, 17 aa, synthetic construct
  REGION 1..17: note = Synthetic Construct
MSWVRQAPGKGLEWVAS

SEQ ID NO: 382 - protein, 8 aa, synthetic construct
  REGION 1..8: note = Synthetic Construct
ISSSGSNT

SEQ ID NO: 383 - protein, 38 aa, synthetic construct
  REGION 1..38: note = Synthetic Construct
YYPDSVKGRFTISRDNAKNNLYLQMNSLRAEDTALYYC

SEQ ID NO: 384 - protein, 11 aa, synthetic construct
  REGION 1..11: note = Synthetic Construct
ARFDYGSSLDS

SEQ ID NO: 385 - protein, 11 aa, synthetic construct
  REGION 1..11: note = Synthetic Construct
WGQGTLLTVSS

SEQ ID NO: 386 - DNA, 321 bp, synthetic construct
  misc_feature 1..321: note = Synthetic Construct
  source 1..321: mol_type = other DNA
gagatcgttcttacccaatccccggatttcctttctgtgacccccaaagaaaaagtcacactcacctgccgagcaagccagtctattagtaacaatttgcactggtatcagcagaagagtgaccaatctcccaaactccttattaagtacgcctctcagtcaatatccggcatacctagccgcttttccggttctggtagtggcaccgactttactctcactatcaattcagtggaggctgaggatgccgccacgtatttttgtcagcaatcaaagagttggccccggacatttggagggggaactaagctggagattaag

SEQ ID NO: 387 - DNA, 78 bp, synthetic construct
  misc_feature 1..78: note = Synthetic Construct
  source 1..78: mol_type = other DNA
gagatcgttcttacccaatccccggatttcctttctgtgacccccaaagaaaaagtcacactcacctgccgagcaagc

SEQ ID NO: 388 - DNA, 18 bp, synthetic construct
  misc_feature 1..18: note = Synthetic Construct
  source 1..18: mol_type = other DNA
cagtctattagtaacaat

SEQ ID NO: 389 - DNA, 51 bp, synthetic construct
  misc_feature 1..51: note = Synthetic Construct
  source 1..51: mol_type = other DNA
ttgcactggtatcagcagaagagtgaccaatctcccaaactccttattaag

SEQ ID NO: 390 - skipped

SEQ ID NO: 391 - DNA, 108 bp, synthetic construct
  misc_feature 1..108: note = Synthetic Construct
  source 1..108: mol_type = other DNA
cagtcaatatccggcatacctagccgcttttccggttctggtagtggcaccgactttactctcactatcaattcagtggaggctgaggatgccgccacgtatttttgt

SEQ ID NO: 392 - DNA, 27 bp, synthetic construct
  misc_feature 1..27: note = Synthetic Construct
  source 1..27: mol_type = other DNA
cagcaatcaaagagttggccccggaca

SEQ ID NO: 393 - DNA, 30 bp, synthetic construct
  misc_feature 1..30: note = Synthetic Construct
  source 1..30: mol_type = other DNA
tttggagggggaactaagctggagattaag

SEQ ID NO: 394 - protein, 107 aa, synthetic construct
  REGION 1..107: note = Synthetic Construct
EIVLTQSPDFLSVTPKEKVTLTCRASQSISNNLHWYQQKSDQSPKLLIKYASQSISGIPSRFSGSGSGTDFTLTINSVEAEDAATYFCQQSKSWPRTFGGGTKLEIK

SEQ ID NO: 395 - protein, 26 aa, synthetic construct
  REGION 1..26: note = Synthetic Construct
EIVLTQSPDFLSVTPKEKVTLTCRAS

SEQ ID NO: 396 - protein, 6 aa, synthetic construct
  REGION 1..6: note = Synthetic Construct
QSISNN

SEQ ID NO: 397 - protein, 17 aa, synthetic construct
  REGION 1..17: note = Synthetic Construct
LHWYQQKSDQSPKLLIK

SEQ ID NO: 398 - skipped

SEQ ID NO: 399 - protein, 36 aa, synthetic construct
  REGION 1..36: note = Synthetic Construct
QSISGIPSRFSGSGSGTDFTLTINSVEAEDAATYFC

SEQ ID NO: 400 - protein, 9 aa, synthetic construct
  REGION 1..9: note = Synthetic Construct
QQSKSWPRT

SEQ ID NO: 401 - protein, 10 aa, synthetic construct
  REGION 1..10: note = Synthetic Construct
FGGGTKLEIK

SEQ ID NO: 402 - DNA, 354 bp, synthetic construct; identical to SEQ ID NO: 370
  misc_feature 1..354: note = Synthetic Construct
  source 1..354: mol_type = other DNA

SEQ ID NO: 403 - DNA, 75 bp, synthetic construct; identical to SEQ ID NO: 371
  misc_feature 1..75: note = Synthetic Construct
  source 1..75: mol_type = other DNA

SEQ ID NO: 404 - DNA, 24 bp, synthetic construct
  misc_feature 1..24: note = Synthetic Construct
  source 1..24: mol_type = other DNA
gggtttacgttctctagttatact

SEQ ID NO: 405 - DNA, 51 bp, synthetic construct; identical to SEQ ID NO: 373
  misc_feature 1..51: note = Synthetic Construct
  source 1..51: mol_type = other DNA

SEQ ID NO: 406 - DNA, 24 bp, synthetic construct
  misc_feature 1..24: note = Synthetic Construct
  source 1..24: mol_type = other DNA
atctctagtagcggcagcaatact

SEQ ID NO: 407 - DNA, 114 bp, synthetic construct; identical to SEQ ID NO: 375
  misc_feature 1..114: note = Synthetic Construct
  source 1..114: mol_type = other DNA

SEQ ID NO: 408 - DNA, 33 bp, synthetic construct; identical to SEQ ID NO: 376
  misc_feature 1..33: note = Synthetic Construct
  source 1..33: mol_type = other DNA

SEQ ID NO: 409 - DNA, 33 bp, synthetic construct; identical to SEQ ID NO: 377
  misc_feature 1..33: note = Synthetic Construct
  source 1..33: mol_type = other DNA

SEQ ID NO: 410 - protein, 118 aa, synthetic construct; identical to SEQ ID NO: 378
  REGION 1..118: note = Synthetic Construct

SEQ ID NO: 411 - protein, 25 aa, synthetic construct
  REGION 1..25: note = Synthetic Construct
EVQLVESGGGLVKPGGSLRLSCAAS

SEQ ID NO: 412 - protein, 8 aa, synthetic construct
  REGION 1..8: note = Synthetic Construct
GFTFSSYT

SEQ ID NO: 413 - protein, 17 aa, synthetic construct
  REGION 1..17: note = Synthetic Construct
MSWVRQAPGKGLEWVAS

SEQ ID NO: 414 - protein, 8 aa, synthetic construct
  REGION 1..8: note = Synthetic Construct
ISSSGSNT

SEQ ID NO: 415 - protein, 38 aa, synthetic construct; identical to SEQ ID NO: 383
  REGION 1..38: note = Synthetic Construct

SEQ ID NO: 416 - protein, 11 aa, synthetic construct
  REGION 1..11: note = Synthetic Construct
ARFDYGSSLDS

SEQ ID NO: 417 - protein, 11 aa, synthetic construct
  REGION 1..11: note = Synthetic Construct
WGQGTLLTVSS

SEQ ID NO: 418 - DNA, 321 bp, synthetic construct
  misc_feature 1..321: note = Synthetic Construct
  source 1..321: mol_type = other DNA
gaaattgtgcttacccagtccccagacttcctgtccgtgacccctaaagagaaggtgacactgacttgcagggcctcacaatccattggcaataaccttcactggtatcagcagaagtccgaccagtctccgaaactcctcatcaagtatgccagccagtcaattagcggaataccgtctcggtttagcggatctgggtctggtactgacttcacgctgacgatcaatagcgtggaagcggaggacgccgccacctatttctgccagcaatctaagtcctggccgagaacgttcggaggcggtactaaacttgagatcaag

SEQ ID NO: 419 - DNA, 78 bp, synthetic construct
  misc_feature 1..78: note = Synthetic Construct
  source 1..78: mol_type = other DNA
gaaattgtgcttacccagtccccagacttcctgtccgtgacccctaaagagaaggtgacactgacttgcagggcctca

SEQ ID NO: 420 - DNA, 18 bp, synthetic construct
  misc_feature 1..18: note = Synthetic Construct
  source 1..18: mol_type = other DNA
caatccattggcaataac

SEQ ID NO: 421 - DNA, 51 bp, synthetic construct
  misc_feature 1..51: note = Synthetic Construct
  source 1..51: mol_type = other DNA
cttcactggtatcagcagaagtccgaccagtctccgaaactcctcatcaag

SEQ ID NO: 422 - skipped

SEQ ID NO: 423 - DNA, 108 bp, synthetic construct
  misc_feature 1..108: note = Synthetic Construct
  source 1..108: mol_type = other DNA
cagtcaattagcggaataccgtctcggtttagcggatctgggtctggtactgacttcacgctgacgatcaatagcgtggaagcggaggacgccgccacctatttctgc

SEQ ID NO: 424 - DNA, 27 bp, synthetic construct
  misc_feature 1..27: note = Synthetic Construct
  source 1..27: mol_type = other DNA
cagcaatctaagtcctggccgagaacg

SEQ ID NO: 425 - DNA, 30 bp, synthetic construct
  misc_feature 1..30: note = Synthetic Construct
  source 1..30: mol_type = other DNA
ttcggaggcggtactaaacttgagatcaag

SEQ ID NO: 426 - protein, 107 aa, synthetic construct
  REGION 1..107: note = Synthetic Construct
EIVLTQSPDFLSVTPKEKVTLTCRASQSIGNNLHWYQQKSDQSPKLLIKYASQSISGIPSRFSGSGSGTDFTLTINSVEAEDAATYFCQQSKSWPRTFGGGTKLEIK

SEQ ID NO: 427 - protein, 26 aa, synthetic construct
  REGION 1..26: note = Synthetic Construct
EIVLTQSPDFLSVTPKEKVTLTCRAS

SEQ ID NO: 428 - protein, 6 aa, synthetic construct
  REGION 1..6: note = Synthetic Construct
QSIGNN

SEQ ID NO: 429 - protein, 17 aa, synthetic construct
  REGION 1..17: note = Synthetic Construct
LHWYQQKSDQSPKLLIK

SEQ ID NO: 430 - skipped

SEQ ID NO: 431 - protein, 36 aa, synthetic construct; identical to SEQ ID NO: 399
  REGION 1..36: note = Synthetic Construct

SEQ ID NO: 432 - protein, 9 aa, synthetic construct
  REGION 1..9: note = Synthetic Construct
QQSKSWPRT

SEQ ID NO: 433 - protein, 10 aa, synthetic construct
  REGION 1..10: note = Synthetic Construct
FGGGTKLEIK

SEQ ID NO: 434 - DNA, 354 bp, synthetic construct
  misc_feature 1..354: note = Synthetic Construct
  source 1..354: mol_type = other DNA
gaggtacagctcgtcgaaagtggcggcggtcttgtcaagccgggaggaagtttgcgcctgtcctgtgcagcatccggattcacgttttcttcttatacgatgagttgggtccggcaggcaccggggaaaggattggaatgggttgcgtctattagtagctctggatctaacacatactacccagactcagttaaaggtcgcttcacgataagtcgggacaacgctaaaaataacctgtatttgcaaatgaacagcttgcgagctgaggacaccgccctctactactgtgcccgatttgattatggatcaagtttggattcatggggccaagggaccctgctcacagtaagctct

SEQ ID NO: 435 - DNA, 75 bp, synthetic construct
  misc_feature 1..75: note = Synthetic Construct
  source 1..75: mol_type = other DNA
gaggtacagctcgtcgaaagtggcggcggtcttgtcaagccgggaggaagtttgcgcctgtcctgtgcagcatcc

SEQ ID NO: 436 - DNA, 24 bp, synthetic construct
  misc_feature 1..24: note = Synthetic Construct
  source 1..24: mol_type = other DNA
ggattcacgttttcttcttatacg

SEQ ID NO: 437 - DNA, 51 bp, synthetic construct
  misc_feature 1..51: note = Synthetic Construct
  source 1..51: mol_type = other DNA
atgagttgggtccggcaggcaccggggaaaggattggaatgggttgcgtct

SEQ ID NO: 438 - DNA, 24 bp, synthetic construct
  misc_feature 1..24: note = Synthetic Construct
  source 1..24: mol_type = other DNA
attagtagctctggatctaacaca

SEQ ID NO: 439 - DNA, 114 bp, synthetic construct
  misc_feature 1..114: note = Synthetic Construct
  source 1..114: mol_type = other DNA
tactacccagactcagttaaaggtcgcttcacgataagtcgggacaacgctaaaaataacctgtatttgcaaatgaacagcttgcgagctgaggacaccgccctctactactgt

SEQ ID NO: 440 - DNA, 33 bp, synthetic construct
  misc_feature 1..33: note = Synthetic Construct
  source 1..33: mol_type = other DNA
gcccgatttgattatggatcaagtttggattca

SEQ ID NO: 441 - DNA, 33 bp, synthetic construct
  misc_feature 1..33: note = Synthetic Construct
  source 1..33: mol_type = other DNA
tggggccaagggaccctgctcacagtaagctct

SEQ ID NO: 442 - protein, 118 aa, synthetic construct; identical to SEQ ID NO: 378
  REGION 1..118: note = Synthetic Construct

SEQ ID NO: 443 - protein, 25 aa, synthetic construct
  REGION 1..25: note = Synthetic Construct
EVQLVESGGGLVKPGGSLRLSCAAS

SEQ ID NO: 444 - protein, 8 aa, synthetic construct
  REGION 1..8: note = Synthetic Construct
GFTFSSYT

SEQ ID NO: 445 - protein, 17 aa, synthetic construct
  REGION 1..17: note = Synthetic Construct
MSWVRQAPGKGLEWVAS

SEQ ID NO: 446 - protein, 8 aa, synthetic construct
  REGION 1..8: note = Synthetic Construct
ISSSGSNT

SEQ ID NO: 447 - protein, 38 aa, synthetic construct; identical to SEQ ID NO: 383
  REGION 1..38: note = Synthetic Construct

SEQ ID NO: 448 - protein, 11 aa, synthetic construct
  REGION 1..11: note = Synthetic Construct
ARFDYGSSLDS

SEQ ID NO: 449 - protein, 11 aa, synthetic construct
  REGION 1..11: note = Synthetic Construct
WGQGTLLTVSS

SEQ ID NO: 450 - DNA, 321 bp, synthetic construct
  misc_feature 1..321: note = Synthetic Construct
  source 1..321: mol_type = other DNA
gaaatcgttcttactcagtccccggattttttgagtgtaacgcctaaagagaaggtgaccctgtcctgccgcgcttcccaatctatatcaaactatcttcattggtaccagcaaaaaagcgaccagtccccgaaactgctcatcaaatacgctagccaatcaataagcggcatccctagcaggttttccggtagcggtagtggcacagacttcacattgagcataaacagcgtggaagccgaggatgcagcaacatacttttgccaacagagcaagtcctggccgaggacgttcggtgggggcaccaaattggaaataaag

SEQ ID NO: 451 - DNA, 78 bp, synthetic construct
  misc_feature 1..78: note = Synthetic Construct
  source 1..78: mol_type = other DNA
gaaatcgttcttactcagtccccggattttttgagtgtaacgcctaaagagaaggtgaccctgtcctgccgcgcttcc

SEQ ID NO: 452 - DNA, 18 bp, synthetic construct
  misc_feature 1..18: note = Synthetic Construct
  source 1..18: mol_type = other DNA
caatctatatcaaactat

SEQ ID NO: 453 - DNA, 51 bp, synthetic construct
  misc_feature 1..51: note = Synthetic Construct
  source 1..51: mol_type = other DNA
cttcattggtaccagcaaaaaagcgaccagtccccgaaactgctcatcaaa

SEQ ID NO: 454 - skipped

SEQ ID NO: 455 - DNA, 108 bp, synthetic construct
  misc_feature 1..108: note = Synthetic Construct
  source 1..108: mol_type = other DNA
caatcaataagcggcatccctagcaggttttccggtagcggtagtggcacagacttcacattgagcataaacagcgtggaagccgaggatgcagcaacatacttttgc

SEQ ID NO: 456 - DNA, 27 bp, synthetic construct
  misc_feature 1..27: note = Synthetic Construct
  source 1..27: mol_type = other DNA
caacagagcaagtcctggccgaggacg

SEQ ID NO: 457 - DNA, 30 bp, synthetic construct
  misc_feature 1..30: note = Synthetic Construct
  source 1..30: mol_type = other DNA
ttcggtgggggcaccaaattggaaataaag

SEQ ID NO: 458 - protein, 107 aa, synthetic construct
  REGION 1..107: note = Synthetic Construct
EIVLTQSPDFLSVTPKEKVTLSCRASQSISNYLHWYQQKSDQSPKLLIKYASQSISGIPSRFSGSGSGTDFTLSINSVEAEDAATYFCQQSKSWPRTFGGGTKLEIK

SEQ ID NO: 459 - protein, 26 aa, synthetic construct
  REGION 1..26: note = Synthetic Construct
EIVLTQSPDFLSVTPKEKVTLSCRAS

SEQ ID NO: 460 - protein, 6 aa, synthetic construct
  REGION 1..6: note = Synthetic Construct
QSISNY

SEQ ID NO: 461 - protein, 17 aa, synthetic construct
  REGION 1..17: note = Synthetic Construct
LHWYQQKSDQSPKLLIK

SEQ ID NO: 462 - skipped

SEQ ID NO: 463 - protein, 36 aa, synthetic construct
  REGION 1..36: note = Synthetic Construct
QSISGIPSRFSGSGSGTDFTLSINSVEAEDAATYFC

SEQ ID NO: 464 - protein, 9 aa, synthetic construct
  REGION 1..9: note = Synthetic Construct
QQSKSWPRT

SEQ ID NO: 465 - protein, 10 aa, synthetic construct
  REGION 1..10: note = Synthetic Construct
FGGGTKLEIK

SEQ ID NO: 466 - DNA, 354 bp, synthetic construct
  misc_feature 1..354: note = Synthetic Construct
  source 1..354: mol_type = other DNA
gaggtccaacttgttgaatccggtggagggctggtgcagcctggtggatccctccgcctttcctgtgcagcatcaggttttactttttcctcatacaccatgtcttgggttcgccaggctccagggaaaggattggaatgggtggcaactatcagtagtagcggggacaatacatactatcccgattccgtgaaagggagatttacgatttcacgcgacaacagcaaaaataccctttacctgcaaatgagttccttgcgggccgaggacactgccctctactactgcgctcgcttcgattacggttccagcctggactcatggggtcaagggactacactgactgtttcttcc

SEQ ID NO: 467 - DNA, 75 bp, synthetic construct
  misc_feature 1..75: note = Synthetic Construct
  source 1..75: mol_type = other DNA
gaggtccaacttgttgaatccggtggagggctggtgcagcctggtggatccctccgcctttcctgtgcagcatca

SEQ ID NO: 468 - DNA, 24 bp, synthetic construct
  misc_feature 1..24: note = Synthetic Construct
  source 1..24: mol_type = other DNA
ggttttactttttcctcatacacc

SEQ ID NO: 469 - DNA, 51 bp, synthetic construct
  misc_feature 1..51: note = Synthetic Construct
  source 1..51: mol_type = other DNA
atgtcttgggttcgccaggctccagggaaaggattggaatgggtggcaact

SEQ ID NO: 470 - DNA, 24 bp, synthetic construct
  misc_feature 1..24: note = Synthetic Construct
  source 1..24: mol_type = other DNA
atcagtagtagcggggacaataca

SEQ ID NO: 471 - DNA, 114 bp, synthetic construct
  misc_feature 1..114: note = Synthetic Construct
  source 1..114: mol_type = other DNA
tactatcccgattccgtgaaagggagatttacgatttcacgcgacaacagcaaaaataccctttacctgcaaatgagttccttgcgggccgaggacactgccctctactactgc

SEQ ID NO: 472 - DNA, 33 bp, synthetic construct
  misc_feature 1..33: note = Synthetic Construct
  source 1..33: mol_type = other DNA
gctcgcttcgattacggttccagcctggactca

SEQ ID NO: 473 - DNA, 33 bp, synthetic construct
  misc_feature 1..33: note = Synthetic Construct
  source 1..33: mol_type = other DNA
tggggtcaagggactacactgactgtttcttcc

SEQ ID NO: 474 - protein, 118 aa, synthetic construct
  REGION 1..118: note = Synthetic Construct
EVQLVESGGGLVQPGGSLRLSCAASGFTFSSYTMSWVRQAPGKGLEWVATISSSGDNTYYPDSVKGRFTISRDNSKNTLYLQMSSLRAEDTALYYCARFDYGSSLDSWGQGTTLTVSS

SEQ ID NO: 475 - protein, 25 aa, synthetic construct [sequence omitted]

SEQ ID NO: 476 - protein, 8 aa, synthetic construct
  REGION 1..8: note = Synthetic Construct
GFTFSSYT

SEQ ID NO: 477 - protein, 17 aa, synthetic construct
  REGION 1..17: note = Synthetic Construct
MSWVRQAPGKGLEWVAT

SEQ ID NO: 478 - protein, 8 aa, synthetic construct
  REGION 1..8: note = Synthetic Construct
ISSSGDNT

SEQ ID NO: 479 - protein, 38 aa, synthetic construct
  REGION 1..38: note = Synthetic Construct
YYPDSVKGRFTISRDNSKNTLYLQMSSLRAEDTALYYC

SEQ ID NO: 480 - protein, 11 aa, synthetic construct
  REGION 1..11: note = Synthetic Construct
ARFDYGSSLDS

SEQ ID NO: 481 - protein, 11 aa, synthetic construct
  REGION 1..11: note = Synthetic Construct
WGQGTTLTVSS

SEQ ID NO: 482 - DNA, 321 bp, synthetic construct
  misc_feature 1..321: note = Synthetic Construct
  source 1..321: mol_type = other DNA
gagatcgtgctcacccaatctcctgacttccttagcgttacaccaggggagaaagtaactcttacgtgccgggcctcccagagcatctccaattatttgcattggtaccagcaaaagagtgaccagagccctaagctgctcatcaaatacgcatcacagagtattagcggcgttccctcacggttctctggctccggttccggtacagacttcactttgacgatttcaagtgtagaggccgaggacttcgcaacttacttttgtcagcaaagcaaatcctggcctcgaactttcggcgggggtacaaaactcgaaatcaag

SEQ ID NO: 483 - DNA, 78 bp, synthetic construct
  misc_feature 1..78: note = Synthetic Construct
  source 1..78: mol_type = other DNA
gagatcgtgctcacccaatctcctgacttccttagcgttacaccaggggagaaagtaactcttacgtgccgggcctcc

SEQ ID NO: 484 - DNA, 18 bp, synthetic construct
  misc_feature 1..18: note = Synthetic Construct
  source 1..18: mol_type = other DNA
cagagcatctccaattat

SEQ ID NO: 485 - DNA, 51 bp, synthetic construct
  misc_feature 1..51: note = Synthetic Construct
  source 1..51: mol_type = other DNA
ttgcattggtaccagcaaaagagtgaccagagccctaagctgctcatcaaa

SEQ ID NO: 486 - skipped

SEQ ID NO: 487 - DNA, 108 bp, synthetic construct
  misc_feature 1..108: note = Synthetic Construct
  source 1..108: mol_type = other DNA
cagagtattagcggcgttccctcacggttctctggctccggttccggtacagacttcactttgacgatttcaagtgtagaggccgaggacttcgcaacttacttttgt

SEQ ID NO: 488 - DNA, 27 bp, synthetic construct
  misc_feature 1..27: note = Synthetic Construct
  source 1..27: mol_type = other DNA
cagcaaagcaaatcctggcctcgaact

SEQ ID NO: 489 - DNA, 30 bp, synthetic construct
  misc_feature 1..30: note = Synthetic Construct
  source 1..30: mol_type = other DNA
ttcggcgggggtacaaaactcgaaatcaag

SEQ ID NO: 490 - protein, 107 aa, synthetic construct
  REGION 1..107: note = Synthetic Construct
EIVLTQSPDFLSVTPGEKVTLTCRASQSISNYLHWYQQKSDQSPKLLIKYASQSISGVPSRFSGSGSGTDFTLTISSVEAEDFATYFCQQSKSWPRTFGGGTKLEIK

SEQ ID NO: 491 - protein, 26 aa, synthetic construct
  REGION 1..26: note = Synthetic Construct
EIVLTQSPDFLSVTPGEKVTLTCRAS

SEQ ID NO: 492 - protein, 6 aa, synthetic construct
  REGION 1..6: note = Synthetic Construct
QSISNY

SEQ ID NO: 493 - protein, 17 aa, synthetic construct
  REGION 1..17: note = Synthetic Construct
LHWYQQKSDQSPKLLIK

SEQ ID NO: 494 - skipped

SEQ ID NO: 495 - protein, 36 aa, synthetic construct
  REGION 1..36: note = Synthetic Construct
QSISGVPSRFSGSGSGTDFTLTISSVEAEDFATYFC

SEQ ID NO: 496 - protein, 9 aa, synthetic construct
  REGION 1..9: note = Synthetic Construct
QQSKSWPRT

SEQ ID NO: 497 - protein, 10 aa, synthetic construct
  REGION 1..10: note = Synthetic Construct
FGGGTKLEIK

SEQ ID NO: 498 - protein, 571 aa, synthetic construct
  REGION 1..571: note = Synthetic Construct
EVQLVESGGGLVKPGGSLRLSCAASGFTFSSYTMSWVRQAPGKGLEWVASISSSGSNTYYPDSVKGRFTISRDNAKNNLYLQMNSLRAEDTALYYCARFDYGSSLDSWGQGTLLTVSSDKTHTEVQLVESGGGLVKPGGSLRLSCAASGFTFSSYTMSWVRQAPGKGLEWVASISSSGSNTYYPDSVKGRFTISRDNAKNNLYLQMNSLRAEDTALYYCARFDYGSSLDSWGQGTLLTVSSDKTHTASTKGPSVFPLAPSSKSTSGGTAALGCLVKDYFPEPVTVSWNSGALTSGVHTFPAVLQSSGSLSSVVTVPSSSLGTQTYICNVNHKPSNTKVDKKVEPKSCDKTHTCPPCPAPELLGGPSVFLFPPKPKDTLYITREPEVTCVVVDVSHEDPEVKFNWYVDGVEVHNAKTKPREEQYNNASRVVSVLTVLHQDWLNGKEYKCKVSNKALPAPIEKTISKAKGQPREPQVYTLPPCRDELTKNQVSLWCLVKGFYPSDIAVEWESNGQPENNYKTTPPVLDSDGSFFKKLTVDKSRWQQGNVFSCSVMHEALHNHYTQKSLSLSPG

SEQ ID NO: 499 - protein, 440 aa, synthetic construct
  REGION 1..440: note = Synthetic Construct
QVQLVQSGAEVVKPGSSVKVSCEASGFTFTDSVITWVRQRPGQGLEWIGEIYPGSGNFYYNEKFQGRVTITADKSTSTAYMELSSLRSEDTAVYFCAMRRSSWGQGTLVTVSSASTKGPSVFPLAPSSKSTSGGTAALGCLVKDYFPEPVTVSWNSGALTSGVHTFPAVLQSSGSLSSVVTVPSSSLGTQTYICNVNHKPSNTKVDKKVEPKSCDKTHTCPPCPAPELLGGPSVFLFPPKPKDTLYITREPEVTCVVVDVSHEDPEVKFNWYVDGVEVHNAKTKPREEQYNNASRVVSVLTVLHQDWLNGKEYKCKVSNKALPAPIEKTISKAKGQPREPQVCTLPPSRDELTKNQVSLSCAVKGFYPSDIAVEWESNGQPENNYKTTPPVLDSDGSFFLVSKLTVDKSRWQQGNVFSCSVMHEALHNRFTQKSLSLSPG

SEQ ID NO: 500 - protein, 331 aa, synthetic construct
  REGION 1..331: note = Synthetic Construct
EIVLTQSPDFLSVTPKEKVTLTCRASQSISNNLHWYQQKSDQSPKLLIKYASQSISGIPSRFSGSGSGTDFTLTINSVEAEDAATYFCQQSKSWPRTFGGGTKLEIKDKTHTEIVLTQSPDFLSVTPKEKVTLTCRASQSISNNLHWYQQKSDQSPKLLIKYASQSISGIPSRFSGSGSGTDFTLTINSVEAEDAATYFCQQSKSWPRTFGGGTKLEIKDKTHTRTVAAPSVFIFPPSDEQLKSGTASVVCLLNNFYPREAKVQWKVDNALQSGNSQESVTEQDSKDSTYSLSSTLTLSKADYEKHKVYACEVTHQGLSSPVTKSFNRGEC

SEQ ID NO: 501 - protein, 219 aa, synthetic construct
  REGION 1..219: note = Synthetic Construct
DVVMTQTPLSLSVTPGQPASISCKSSQTIVHSNSKTYLEWYLQKPGQSPQLLIYKVSSRFSGVPDRFSGSGSGTDFTLKISRVEAEDVGVYYCFQGSHVPLTFGQGTKLEIKRTVAAPSVFIFPPSDEQLKSGTASVVCLLNNFYPREAKVQWKVDNALQSGNSQESVTEQDSKDSTYSLSSTLTLSKADYEKHKVYACEVTHQGLSSPVTKSFNRGEC

SEQ ID NO: 502 - protein, 571 aa, synthetic construct; identical to SEQ ID NO: 498
  REGION 1..571: note = Synthetic Construct

SEQ ID NO: 503 - protein, 440 aa, synthetic construct; identical to SEQ ID NO: 499
  REGION 1..440: note = Synthetic Construct

SEQ ID NO: 504 - protein, 331 aa, synthetic construct
  REGION 1..331: note = Synthetic Construct
EIVLTQSPDFLSVTPKEKVTLSCRASQSISNYLHWYQQKSDQSPKLLIKYASQSISGIPSRFSGSGSGTDFTLSINSVEAEDAATYFCQQSKSWPRTFGGGTKLEIKDKTHTEIVLTQSPDFLSVTPKEKVTLTCRASQSISNNLHWYQQKSDQSPKLLIKYASQSISGIPSRFSGSGSGTDFTLTINSVEAEDAATYFCQQSKSWPRTFGGGTKLEIKDKTHTRTVAAPSVFIFPPSDEQLKSGTASVVCLLNNFYPREAKVQWKVDNALQSGNSQESVTEQDSKDSTYSLSSTLTLSKADYEKHKVYACEVTHQGLSSPVTKSFNRGEC

SEQ ID NO: 505 - protein, 219 aa, synthetic construct; identical to SEQ ID NO: 501
  REGION 1..219: note = Synthetic Construct

SEQ ID NO: 506 - protein, 571 aa, synthetic construct
  REGION 1..571: note = Synthetic Construct
EVQLVESGGGLVKPGGSLRLSCAASGFTFSSYTMSWVRQAPGKGLEWVASISSSGSNTYYPDSVKGRFTISRDNAKNNLYLQMNSLRAEDTALYYCARFDYGSSLDSWGQGTLLTVSSDKTHTEVQLVESGGGLVQPGGSLRLSCAASGFTFSSYTMSWVRQAPGKGLEWVATISSSGDNTYYPDSVKGRFTISRDNSKNTLYLQMSSLRAEDTALYYCARFDYGSSLDSWGQGTTLTVSSDKTHTASTKGPSVFPLAPSSKSTSGGTAALGCLVKDYFPEPVTVSWNSGALTSGVHTFPAVLQSSGSLSSVVTVPSSSLGTQTYICNVNHKPSNTKVDKKVEPKSCDKTHTCPPCPAPELLGGPSVFLFPPKPKDTLYITREPEVTCVVVDVSHEDPEVKFNWYVDGVEVHNAKTKPREEQYNNASRVVSVLTVLHQDWLNGKEYKCKVSNKALPAPIEKTISKAKGQPREPQVYTLPPCRDELTKNQVSLWCLVKGFYPSDIAVEWESNGQPENNYKTTPPVLDSDGSFFKKLTVDKSRWQQGNVFSCSVMHEALHNHYTQKSLSLSPG

SEQ ID NO: 507 - protein, 440 aa, synthetic construct; identical to SEQ ID NO: 499
  REGION 1..440: note = Synthetic Construct

SEQ ID NO: 508 - protein, 331 aa, synthetic construct
  REGION 1..331: note = Synthetic Construct
EIVLTQSPDFLSVTPGEKVTLTCRASQSISNYLHWYQQKSDQSPKLLIKYASQSISGVPSRFSGSGSGTDFTLTISSVEAEDFATYFCQQSKSWPRTFGGGTKLEIKDKTHTEIVLTQSPDFLSVTPKEKVTLTCRASQSIGNNLHWYQQKSDQSPKLLIKYASQSISGIPSRFSGSGSGTDFTLTINSVEAEDAATYFCQQSKSWPRTFGGGTKLEIKDKTHTRTVAAPSVFIFPPSDEQLKSGTASVVCLLNNFYPREAKVQWKVDNALQSGNSQESVTEQDSKDSTYSLSSTLTLSKADYEKHKVYACEVTHQGLSSPVTKSFNRGEC

SEQ ID NO: 509 - protein, 219 aa, synthetic construct; identical to SEQ ID NO: 501
  REGION 1..219: note = Synthetic Construct

SEQ ID NO: 510 - protein, 571 aa, synthetic construct; identical to SEQ ID NO: 498
  REGION 1..571: note = Synthetic Construct

SEQ ID NO: 511 - protein, 440 aa, synthetic construct; identical to SEQ ID NO: 499
  REGION 1..440: note = Synthetic Construct

SEQ ID NO: 512 - protein, 331 aa, synthetic construct
  REGION 1..331: note = Synthetic Construct
EIVLTQSPDFLSVTPKEKVTLTCRASQSIGNNLHWYQQKSDQSPKLLIKYASQSISGIPSRFSGSGSGTDFTLTINSVEAEDAATYFCQQSKSWPRTFGGGTKLEIKDKTHTEIVLTQSPDFLSVTPKEKVTLSCRASQSISNYLHWYQQKSDQSPKLLIKYASQSISGIPSRFSGSGSGTDFTLSINSVEAEDAATYFCQQSKSWPRTFGGGTKLEIKDKTHTRTVAAPSVFIFPPSDEQLKSGTASVVCLLNNFYPREAKVQWKVDNALQSGNSQESVTEQDSKDSTYSLSSTLTLSKADYEKHKVYACEVTHQGLSSPVTKSFNRGEC

SEQ ID NO: 513 - protein, 219 aa, synthetic construct; identical to SEQ ID NO: 501
  REGION 1..219: note = Synthetic Construct

SEQ ID NO: 514 - protein, 571 aa, synthetic construct
  REGION 1..571: note = Synthetic Construct
EVQLVESGGGLVQPGGSLRLSCAASGFTFSSYTMSWVRQAPGKGLEWVATISSSGDNTYYPDSVKGRFTISRDNSKNTLYLQMSSLRAEDTALYYCARFDYGSSLDSWGQGTTLTVSSDKTHTEVQLVESGGGLVKPGGSLRLSCAASGFTFSSYTMSWVRQAPGKGLEWVASISSSGSNTYYPDSVKGRFTISRDNAKNNLYLQMNSLRAEDTALYYCARFDYGSSLDSWGQGTLLTVSSDKTHTASTKGPSVFPLAPSSKSTSGGTAALGCLVKDYFPEPVTVSWNSGALTSGVHTFPAVLQSSGSLSSVVTVPSSSLGTQTYICNVNHKPSNTKVDKKVEPKSCDKTHTCPPCPAPELLGGPSVFLFPPKPKDTLYITREPEVTCVVVDVSHEDPEVKFNWYVDGVEVHNAKTKPREEQYNNASRVVSVLTVLHQDWLNGKEYKCKVSNKALPAPIEKTISKAKGQPREPQVYTLPPCRDELTKNQVSLWCLVKGFYPSDIAVEWESNGQPENNYKTTPPVLDSDGSFFKKLTVDKSRWQQGNVFSCSVMHEALHNHYTQKSLSLSPG

SEQ ID NO: 515 - protein, 440 aa, synthetic construct; identical to SEQ ID NO: 499
  REGION 1..440: note = Synthetic Construct

SEQ ID NO: 516 - protein, 331 aa, synthetic construct
  REGION 1..331: note = Synthetic Construct
EIVLTQSPDFLSVTPKEKVTLTCRASQSISNNLHWYQQKSDQSPKLLIKYASQSISGIPSRFSGSGSGTDFTLTINSVEAEDAATYFCQQSKSWPRTFGGGTKLEIKDKTHTEIVLTQSPDFLSVTPGEKVTLTCRASQSISNYLHWYQQKSDQSPKLLIKYASQSISGVPSRFSGSGSGTDFTLTISSVEAEDFATYFCQQSKSWPRTFGGGTKLEIKDKTHTRTVAAPSVFIFPPSDEQLKSGTASVVCLLNNFYPREAKVQWKVDNALQSGNSQESVTEQDSKDSTYSLSSTLTLSKADYEKHKVYACEVTHQGLSSPVTKSFNRGEC

SEQ ID NO: 517 - protein, 219 aa, synthetic construct; identical to SEQ ID NO: 501
  REGION 1..219: note = Synthetic Construct

SEQ ID NO: 518 - protein, 438 aa, synthetic construct
  REGION 1..438: note = Synthetic Construct
QVQLVQSGAEVVKPGSSVKVSCEASGFTFTDSVITWVRQRPGQGLEWIGEIYPGSGNFYYNEKFQGRVTITADKSTSTAYMELSSLRSEDTAVYFCAMRRSSWGQGTLVTVSSASTKGPSVFPLAPSSKSTSGGTAALGCLVKDYFPEPVTVSWNSGALTSGVHTFPAVLQSSGSLSSVVTVPSSSLGTQTYICNVNHKPSNTKVDKKVEPKSCDKTHTCPPCPAPELLGGPSVFLFPPKPKDTLMISRTPEVTCVVVDVSHEDPEVKFNWYVDGVEVHNAKTKPREEQYNNASRVVSVLTVLHQDWLNGKEYKCKVSNKALPAPIEKTISKAKGQPREPQVYTLPPSRDELTKNQVSLTCLVKGFYPSDIAVEWESNGQPENNYKTTPPVLDSDGSFFKRLTVDKSRWQQGNVFSCSVMHEALHNHYTQKSLSLSPG

SEQ ID NO: 519 - protein, 443 aa, synthetic construct
  REGION 1..443: note = Synthetic Construct
EVQLVESGGGLVKPGGSLRLSCAASGFTFSSYTMSWVRQAPGKGLEWVASISSSGSNTYYPDSVKGRFTISRDNAKNNLYLQMNSLRAEDTALYYCARFDYGSSLDSWGQGTLLTVSSASTKGPSVFPLAPSSKSTSGGTAALGCLVKDYFPEPVTVSWNSGALTSGVHTFPAVLQSSGSLSSVVTVPSSSLGTQTYICNVNHKPSNTKVDKKVEPKSCDKTHTCPPCPAPELLGGPSVFLFPPKPKDTLMISRTPEVTCVVVDVSHEDPEVKFNWYVDGVEVHNAKTKPREEQYNNSARVVSVLTVLHQDWLNGKEYKCKVSNKALPAPIEKTISKAKGQPREPQVYTLPPSRDELTKNQVSLTCLVKGFYPSDIAVEWESNGQPENNYKTTPPVLDSDGSFLKKLTVDKSRWQQGNVFSCSVMHEALHNHYTQKSLSLSPG

SEQ ID NO: 520 - protein, 219 aa, synthetic construct; identical to SEQ ID NO: 501
  REGION 1..219: note = Synthetic Construct

SEQ ID NO: 521 - protein, 214 aa, synthetic construct
  REGION 1..214: note = Synthetic Construct
EIVLTQSPDFLSVTPKEKVTLTCRASQSISNNLHWYQQKSDQSPKLLIKYASQSISGIPSRFSGSGSGTDFTLTINSVEAEDAATYFCQQSKSWPRTFGGGTKLEIKRTVAAPSVFIFPPSDEQLKSGTASVVCLLNNFYPREAKVQWKVDNALQSGNSQESVTEQDSKDSTYSLSSTLTLSKADYEKHKVYACEVTHQGLSSPVTKSFNRGEC

SEQ ID NO: 522 - protein, 566 aa, synthetic construct
  REGION 1..566: note = Synthetic Construct
QVQLVQSGAEVVKPGSSVKVSCEASGFTFTDSVITWVRQRPGQGLEWIGEIYPGSGNFYYNEKFQGRVTITADKSTSTAYMELSSLRSEDTAVYFCAMRRSSWGQGTLVTVSSGGGGSGGGGSEVQLVESGGGLVKPGGSLRLSCAASGFTFSSYTMSWVRQAPGKGLEWVASISSSGSNTYYPDSVKGRFTISRDNAKNNLYLQMNSLRAEDTALYYCARFDYGSSLDSWGQGTLLTVSSASTKGPSVFPLAPSSKSTSGGTAALGCLVKDYFPEPVTVSWNSGALTSGVHTFPAVLQSSGSLSSVVTVPSSSLGTQTYICNVNHKPSNTKVDKKVEPKSCDKTHTCPPCPAPELLGGPSVFLFPPKPKDTLMISRTPEVTCVVVDVSHEDPEVKFNWYVDGVEVHNAKTKPREEQYNNASRVVSVLTVLHQDWLNGKEYKCKVSNKALPAPIEKTISKAKGQPREPQVYTLPPSRDELTKNQVSLTCLVKGFYPSDIAVEWESNGQPENNYKTTPPVLDSDGSFFKKLTVDKSRWQQGNVFSCSVMHEALHNHYTQKSLSLSPG

SEQ ID NO: 523 - protein, 336 aa, synthetic construct
  REGION 1..336: note = Synthetic Construct
DVVMTQTPLSLSVTPGQPASISCKSSQTIVHSNSKTYLEWYLQKPGQSPQLLIYKVSSRFSGVPDRFSGSGSGTDFTLKISRVEAEDVGVYYCFQGSHVPLTFGQGTKLEIKGGGGSGGGGSEIVLTQSPDFLSVTPKEKVTLTCRASQSISNNLHWYQQKSDQSPKLLIKYASQSISGIPSRFSGSGSGTDFTLTINSVEAEDAATYFCQQSKSWPRTFGGGTKLEIKRTVAAPSVFIFPPSDEQLKSGTASVVCLLNNFYPREAKVQWKVDNALQSGNSQESVTEQDSKDSTYSLSSTLTLSKADYEKHKVYACEVTHQGLSSPVTKSFNRGEC

SEQ ID NO: 524 - protein, 438 aa, synthetic construct
  REGION 1..438: note = Synthetic Construct
QVQLVQSGAEVVKPGSSVKVSCEASGFTFTDSVITWVRQRPGQGLEWIGEIYPGSGNFYYNEKFQGRVTITADKSTSTAYMELSSLRSEDTAVYFCAMRRSSWGQGTLVTVSSASTKGPSVCPLAPSSKSTSGGTAALGCLVKDYFPEPVTVSWNSGALTSGVHTFPAVLQSSGSLSSVVTVPSSSLGTQTYICNVNHKPSNTKVDKKVEPKSVDKTHTCPPCPAPELLGGPSVFLFPPKPKDTLMISRTPEVTCVVVDVSHEDPEVKFNWYVDGVEVHNAKTKPREEQYNNASRVVSVLTVLHQDWLNGKEYKCKVSNKALPAPIEKTISKAKGQPREPQVYTLPPCRDELTKNQVSLWCLVKGFYPSDIAVEWESNGQPENNYKTTPPVLDSDGSFFKKLTVDKSRWQQGNVFSCSVMHEALHNHYTQKSLSLSPG

SEQ ID NO: 525 - protein, 445 aa, synthetic construct
  REGION 1..445: note = Synthetic Construct
EVQLVESGGGLVKPGGSLRLSCAASGFTFSSYTMSWVRQAPGKGLEWVASISSSGSNTYYPDSVKGRFTISRDNAKNNLYLQMNSLRAEDTALYYCARFDYGSSLDSWGQGTLLTVSSASTKGPSVFPLAPSSKSTSGGTAALGCLVKDYFPEPVTVSWNSGALTSGVHTFPAVLQSSGSLSSVVTVPSSSLGTQTYICNVNHKPSNTKVDKKVEPKSCDKTHTCPPCPAPELLGGPSVFLFPPKPKDTLMISRTPEVTCVVVDVSHEDPEVKFNWYVDGVEVHNAKTKPREEQYNNASRVVSVLTVLHQDWLNGKEYKCKVSNKALPAPIEKTISKAKGQPREPQVCTLPPSRDELTKNQVSLSCAVKGFYPSDIAVEWESNGQPENNYKTTPPVLDSDGSFFLVSKLTVDKSRWQQGNVFSCSVMHEALHNRFTQKSLSLSPG

SEQ ID NO: 526 - protein, 219 aa, synthetic construct
  REGION 1..219: note = Synthetic Construct
DVVMTQTPLSLSVTPGQPASISCKSSQTIVHSNSKTYLEWYLQKPGQSPQLLIYKVSSRFSGVPDRFSGSGSGTDFTLKISRVEAEDVGVYYCFQGSHVPLTFGQGTKLEIKRTVAAPSVFIFPPCDEQLKSGTASVVCLLNNFYPREAKVQWKVDNALQSGNSQESVTEQDSKDSTYSLSSTLTLSKADYEKHKVYACEVTHQGLSSPVTKSFNRGEV

SEQ ID NO: 527 - protein, 214 aa, synthetic construct
  REGION 1..214: note = Synthetic Construct
EIVLTQSPDFLSVTPKEKVTLSCRASQSISNYLHWYQQKSDQSPKLLIKYASQSISGIPSRFSGSGSGTDFTLSINSVEAEDAATYFCQQSKSWPRTFGGGTKLEIKRTVAAPSVFIFPPSDEQLKSGTASVVCLLNNFYPREAKVQWKVDNALQSGNSQESVTEQDSKDSTYSLSSTLTLSKADYEKHKVYACEVTHQGLSSPVTKSFNRGEC

SEQ ID NO: 528 - protein, 566 aa, synthetic construct; identical to SEQ ID NO: 522
  REGION 1..566: note = Synthetic Construct

SEQ ID NO: 529 - protein, 336 aa, synthetic construct
  REGION 1..336: note = Synthetic Construct
DVVMTQTPLSLSVTPGQPASISCKSSQTIVHSNSKTYLEWYLQKPGQSPQLLIYKVSSRFSGVPDRFSGSGSGTDFTLKISRVEAEDVGVYYCFQGSHVPLTFGQGTKLEIKGGGGSGGGGSEIVLTQSPDFLSVTPKEKVTLSCRASQSISNYLHWYQQKSDQSPKLLIKYASQSISGIPSRFSGSGSGTDFTLSINSVEAEDAATYFCQQSKSWPRTFGGGTKLEIKRTVAAPSVFIFPPSDEQLKSGTASVVCLLNNFYPREAKVQWKVDNALQSGNSQESVTEQDSKDSTYSLSSTLTLSKADYEKHKVYACEVTHQGLSSPVTKSFNRGEC

SEQ ID NO: 530 - protein, 559 aa, synthetic construct
  REGION 1..559: note = Synthetic Construct
QVQLVQSGAEVVKPGSSVKVSCEASGFTFTDSVITWVRQRPGQGLEWIGEIYPGSGNFYYNEKFQGRVTITADKSTSTAYMELSSLRSEDTAVYFCAMRRSSWGQGTLVTVSSSEVQLVESGGGLVKPGGSLRLSCAASGFTFSSYTMSWVRQAPGKGLEWVASISSSGSNTYYPDSVKGRFTISRDNAKNNLYLQMNSLRAEDTALYYCARFDYGSSLDSWGQGTLLTVSSRTASTKGPSVFPLAPSSKSTSGGTAALGCLVKDYFPEPVTVSWNSGALTSGVHTFPAVLQSSGSLSSVVTVPSSSLGTQTYICNVNHKPSNTKVDKKVEPKSCDKTHTCPPCPAPELLGGPSVFLFPPKPKDTLMISRTPEVTCVVVDVSHEDPEVKFNWYVDGVEVHNAKTKPREEQYNNASRVVSVLTVLHQDWLNGKEYKCKVSNKALPAPIEKTISKAKGQPREPQVYTLPPSRDELTKNQVSLTCLVKGFYPSDIAVEWESNGQPENNYKTTPPVLDSDGSFFKKLTVDKSRWQQGNVFSCSVMHEALHNHYTQKSLSLSPG

SEQ ID NO: 531 - protein, 338 aa, synthetic construct
  REGION 1..338: note = Synthetic Construct
EIVLTQSPDFLSVTPKEKVTLTCRASQSIGNNLHWYQQKSDQSPKLLIKYASQSISGIPSRFSGSGSGTDFTLTINSVEAEDAATYFCQQSKSWPRTFGGGTKLEIKGQPKAAPDVVMTQTPLSLSVTPGQPASISCRSSQTIVHSNSKTYLEWYLQKPGQSPQLLIYKVSNRFSGVPDRFSGSGSGTDFTLKISRVEAEDVGVYYCFQGSHVPLTFGAGTKLEIKTKGPSRTVAAPSVFIFPPSDEQLKSGTASVVCLLNNFYPREAKVQWKVDNALQSGNSQESVTEQDSKDSTYSLSSTLTLSKADYEKHKVYACEVTHQGLSSPVTKSFNRGEC

SEQ ID NO: 532 - protein, 559 aa, synthetic construct
  REGION 1..559: note = Synthetic Construct
QVQLVQSGAEVVKPGSSVKVSCEASGFTFTDSVITWVRQRPGQGLEWIGEIYPGSGNFYYNEKFQGRVTITADKSTSTAYMELSSLRSEDTAVYFCAMRRSSWGQGTLVTVSSSEVQLVESGGGLVQPGGSLRLSCAASGFTFSSYTMSWVRQAPGKGLEWVATISSSGDNTYYPDSVKGRFTISRDNSKNTLYLQMSSLRAEDTALYYCARFDYGSSLDSWGQGTTLTVSSRTASTKGPSVFPLAPSSKSTSGGTAALGCLVKDYFPEPVTVSWNSGALTSGVHTFPAVLQSSGSLSSVVTVPSSSLGTQTYICNVNHKPSNTKVDKKVEPKSCDKTHTCPPCPAPELLGGPSVFLFPPKPKDTLMISRTPEVTCVVVDVSHEDPEVKFNWYVDGVEVHNAKTKPREEQYNNASRVVSVLTVLHQDWLNGKEYKCKVSNKALPAPIEKTISKAKGQPREPQVYTLPPSRDELTKNQVSLTCLVKGFYPSDIAVEWESNGQPENNYKTTPPVLDSDGSFFKKLTVDKSRWQQGNVFSCSVMHEALHNHYTQKSLSLSPG

SEQ ID NO: 533 - protein, 338 aa, synthetic construct
  REGION 1..338: note = Synthetic Construct
EIVLTQSPDFLSVTPGEKVTLTCRASQSISNYLHWYQQKSDQSPKLLIKYASQSISGVPSRFSGSGSGTDFTLTISSVEAEDFATYFCQQSKSWPRTFGGGTKLEIKGQPKAAPDVVMTQTPLSLSVTPGQPASISCRSSQTIVHSNSKTYLEWYLQKPGQSPQLLIYKVSNRFSGVPDRFSGSGSGTDFTLKISRVEAEDVGVYYCFQGSHVPLTFGAGTKLEIKTKGPSRTVAAPSVFIFPPSDEQLKSGTASVVCLLNNFYPREAKVQWKVDNALQSGNSQESVTEQDSKDSTYSLSSTLTLSKADYEKHKVYACEVTHQGLSSPVTKSFNRGEC

SEQ ID NO: 534 - protein, 5 aa, synthetic construct
  REGION 1..5: note = Synthetic Construct
DKTHT